European Patent Application EP 4 286 401 A1, published December 6, 2023. Title: USE OF AN ARTIFICIAL PROTEIN OR OF A NUCLEIC ACID ENCODING THE ARTIFICIAL PROTEIN FOR PROVIDING A FUNCTIONAL RIBONUCLEOPROTEIN COMPLEX. Applicant: Technische Universität Dresden. The sequence listing filed with the application follows.

SEQUENCE LISTING (86 sequences)

SEQ ID NO: 1 - protein, 8 aa, artificial sequence
  core consensus amino acid sequence of 2A peptides
  NON_STD 2..2: Xaa can be any naturally occurring amino acid
  NON_STD 4..4: Xaa can be any naturally occurring amino acid
DXEXNPGP

SEQ ID NO: 2 - protein, 5 aa, artificial sequence
  Motif of linker
GGGGS

SEQ ID NO: 3 - protein, 18 aa, artificial sequence
  Motif of linker
KESGSVSSEQLAQFRSLE

SEQ ID NO: 4 - protein, 18 aa, artificial sequence
  Motif of linker
KESGSVSSEQLAQFRSLD

SEQ ID NO: 5 - protein, 14 aa, artificial sequence
  Motif of linker
EGKSSGSGSESKST

SEQ ID NO: 6 - protein, 5 aa, artificial sequence
  Motif of linker
EAAAK

SEQ ID NO: 7 - protein, 6 aa, artificial sequence
  Motif of linker
LPEPEP

SEQ ID NO: 8 - protein, 7 aa, artificial sequence
  SV40 NLS
PKKKRKV

SEQ ID NO: 9 - protein, 16 aa, artificial sequence
  nucleoplasmin NLS
KRPAATKKAGQAKKKK

SEQ ID NO: 10 - protein, 18 aa, artificial sequence
  SV40 bipartite NLS
KRTADGSEFESPKKKRKV

SEQ ID NO: 11 - RNA, 20 nt, artificial sequence
  Csy4 cleavage sequence
guucacugccguauaggcag

SEQ ID NO: 12 - RNA, 28 nt, artificial sequence
  Csy4 cleavage sequence
guucacugccguauaggcagcuaagaaa

SEQ ID NO: 13 - RNA, 20 nt, artificial sequence
  Csy4 cleavage sequence
guacacugccguauaggcag

SEQ ID NO: 14 - RNA, 20 nt, artificial sequence
  Csy4 cleavage sequence
guaaacugccguauaggcag

SEQ ID NO: 15 - RNA, 20 nt, artificial sequence
  Csy4 cleavage sequence
guucccugccguauaggcag

SEQ ID NO: 16 - DNA, 23 bp, artificial sequence
  stuffer C9-sgRNA targeting sequence with PAM
  misc_feature 21..21: /note="n is a, c, g, or t"
cgagacgagcttgcgtctcgngg

SEQ ID NO: 17 - DNA, 23 bp, artificial sequence
  gfp-148 C9-sgRNA targeting sequence with PAM
gggcacgggcagcttgccggtgg

SEQ ID NO: 18 - DNA, 23 bp, artificial sequence
  gfp-197 C9-sgRNA targeting sequence with PAM
gctgaagcactgcacgccgtagg

SEQ ID NO: 19 - DNA, 23 bp, artificial sequence
  gfp-112 C9-sgRNA targeting sequence with PAM
cagggtcagcttgccgtaggtgg

SEQ ID NO: 20 - DNA, 23 bp, artificial sequence
  gfp+174 C9-sgRNA targeting sequence with PAM
ccggcaagctgcccgtgccctgg

SEQ ID NO: 21 - DNA, 25 bp, artificial sequence
  gfp c.187 A>G C9-sgRNA targeting sequence with PAM
gccgtaggtcagggtggtcacgagg

SEQ ID NO: 22 - DNA, 23 bp, artificial sequence
  sgTRAC1 C9-sgRNA targeting sequence with PAM
gcagggttctggatatctgtggg

SEQ ID NO: 23 - DNA, 24 bp, artificial sequence
  sgTRAC3 C9-sgRNA targeting sequence with PAM
gagagtctctcagctggtacacgg

SEQ ID NO: 24 - DNA, 20 bp, artificial sequence
  Cas9 forward primer
ggaccaggaactggacatca

SEQ ID NO: 25 - DNA, 20 bp, artificial sequence
  Cas9 reverse primer
tcgatggagtcgtccttcag

SEQ ID NO: 26 - DNA, 24 bp, artificial sequence
  Cas9 probe
  misc_binding 1: /note="fluorescein (FAM)"
  misc_binding 24: /note="black hole quencher 1 (BHQ1)"
ccacatcgtagtcggacagccggt

SEQ ID NO: 27 - DNA, 20 bp, artificial sequence
  pre-C4/C9-sgRNA forward primer
cggtgcgttcactgccgtat

SEQ ID NO: 28 - DNA, 21 bp, artificial sequence
  pre-C4/C9-sgRNA reverse primer
agcagcgtatccacatagcgt

SEQ ID NO: 29 - DNA, 20 bp, artificial sequence
  pre-C4/C9-sgRNA probe
  misc_binding 1: /note="ATTO 550 fluorescent label"
  misc_binding 20: /note="black hole quencher 2 (BHQ2)"
ttgtcgacgcggccgctgcc

SEQ ID NO: 30 - DNA, 24 bp, artificial sequence
  C9-sgRNA forward primer
gttttagagctagaaatagcaagt

SEQ ID NO: 31 - DNA, 19 bp, artificial sequence
  C9-sgRNA reverse primer
ccgactcggtgccactttt

SEQ ID NO: 32 - DNA, 19 bp, artificial sequence
  C9-sgRNA probe
  misc_binding 1: /note="fluorescein (FAM)"
  misc_binding 19: /note="minor groove binder (MGB)"
acggactagccttatttta

SEQ ID NO: 33 - protein, 18 aa, artificial sequence
  T2A peptide
EGRGSLLTCGDVEENPGP

SEQ ID NO: 34 - protein, 36 aa, artificial sequence
  Linker sequence of C4C9v1
FEGGGGSGGGGSGGGGSARMAPKKKRKVGIHGVPAA

SEQ ID NO: 35 - protein, 42 aa, artificial sequence
  Linker sequence of C9C4v1
KRPAATKKAGQAKKKKASGSGLQFEGGGGSGGGGSGGGGSAS

SEQ ID NO: 36 - protein, 39 aa, artificial sequence
  Linker sequence of C4C9v2, C4C9v2-1
FEGGGGSGGGGSGGGGSGGGGSGGGGSGGGGSGGGGSGT

SEQ ID NO: 37 - protein, 19 aa, artificial sequence
  Linker sequence of C4C9v3
FEGGGGSGGGGSGGGGSGT

SEQ ID NO: 38 - protein, 40 aa, artificial sequence
  Linker sequence of C9C4v2, C9C4v2-1, C9C4v2 BE1
NCLGGGGSGGGGSGGGGSGGGGSGGGGSGGGGSGGGGSTG

SEQ ID NO: 39 - protein, 20 aa, artificial sequence
  Linker sequence of C9C4v3
NCLGGGGSGGGGSGGGGSTG

SEQ ID NO: 40 - DNA, 67 bp, artificial sequence
  scrambled shRNA
gaaacaccggcaacaagatgaagagcaccaagttaatattcatagcttggtgctcttcatcttgttg

SEQ ID NO: 41 - DNA, 57 bp, artificial sequence
  C4-688 shRNA
gaaggaggctttacttgttatgttaatattcatagcataacaagtaaagcctccttc

SEQ ID NO: 42 - DNA, 57 bp, artificial sequence
  sgRNA-947 shRNA
gagctagaaatagcaagttaagttaatattcatagcttaacttgctatttctagctc

SEQ ID NO: 43 - DNA, 29 bp, artificial sequence
  complementary sequence to sequence comprising gfp-148 sgRNA targeting sequence
gcaccaccggcaagctgcccgtgccctgg

SEQ ID NO: 44 - protein, 9 aa, artificial sequence
  portion of GFP
TTGKLPVPW

SEQ ID NO: 45 - DNA, 29 bp, artificial sequence
  sequence comprising gfp-148 sgRNA targeting sequence
ccagggcacgggcagcttgccggtggtgc

SEQ ID NO: 46 - RNA, 20 nt, artificial sequence
  gfp-148 sgRNA
gggcacgggcagcuugccgg

SEQ ID NO: 47 - DNA, 31 bp, artificial sequence
  complementary sequence to sequence comprising gfp c.187 A>G sgRNA targeting sequence
caccctcgtgaccaccctgacctacggcgtg

SEQ ID NO: 48 - protein, 10 aa, artificial sequence
  portion of GFP
TLVTTLTYGV

SEQ ID NO: 49 - DNA, 31 bp, artificial sequence
  sequence comprising gfp c.187 A>G sgRNA targeting sequence
cacgccgtaggtcagggtggtcacgagggtg

SEQ ID NO: 50 - RNA, 22 nt, artificial sequence
  gfp c.187 A>G sgRNA
gccguaggucaggguggucacg

SEQ ID NO: 51 - protein, 1609 aa, artificial sequence
  artificial protein C4C9v1
MGDHYLDIRLRPDPEFPPAQLMSVLFGKLHQALVAQGGDRIGVSFPDLDESRSRLGERLRIHASADDLRALLARPWLEGLRDHLQFGEPAVVPHPTPYRQVSRVQAKSNPERLRRRLMRRHDLSEEEARKRIPDTVARALDLPFVTLRSQSTGQHFRLFIRHGPLQVTAEEGGFTCYGLSKGGFVPWFFEGGGGSGGGGSGGGGSARMAPKKKRKVGIHGVPAADKKYSIGLDIGTNSVGWAVITDEYKVPSKKFKVLGNTDRHSIKKNLIGALLFDSGETAEATRLKRTARRRYTRRKNRICYLQEIFSNEMAKVDDSFFHRLEESFLVEEDKKHERHPIFGNIVDEVAYHEKYPTIYHLRKKLVDSTDKADLRLIYLALAHMIKFRGHFLIEGDLNPDNSDVDKLFIQLVQTYNQLFEENPINASGVDAKAILSARLSKSRRLENLIAQLPGEKKNGLFGNLIALSLGLTPNFKSNFDLAEDAKLQLSKDTYDDDLDNLLAQIGDQYADLFLAAKNLSDAILLSDILRVNTEITKAPLSASMIKRYDEHHQDLTLLKALVRQQLPEKYKEIFFDQSKNGYAGYIDGGASQEEFYKFIKPILEKMDGTEELLVKLNREDLLRKQRTFDNGSIPHQIHLGELHAILRRQEDFYPFLKDNREKIEKILTFRIPYYVGPLARGNSRFAWMTRKSEETITPWNFEEVVDKGASAQSFIERMTNFDKNLPNEKVLPKHSLLYEYFTVYNELTKVKYVTEGMRKPAFLSGEQKKAIVDLLFKTNRKVTVKQLKEDYFKKIECFDSVEISGVEDRFNASLGTYHDLLKIIKDKDFLDNEENEDILEDIVLTLTLFEDREMIEERLKTYAHLFDDKVMKQLKRRRYTGWGRLSRKLINGIRDKQSGKTILDFLKSDGFANRNFMQLIHDDSLTFKEDIQKAQVSGQGDSLHEHIANLAGSPAIKKGILQTVKVVDELVKVMGRHKPENIVIEMARENQTTQKGQKNSRERMKRIEEGIKELGSQILKEHPVENTQLQNEKLYLYYLQNGRDMYVDQELDINRLSDYDVDHIVPQSFLKDDSIDNKVLTRSDKNRGKSDNVPSEEVVKKMKNYWRQLLNAKLITQRKFDNLTKAERGGLSELDKAGFIKRQLVETRQITKHVAQILDSRMNTKYDENDKLIREVKVITLKSKLVSDFRKDFQFYKVREINNYHHAHDAYLNAVVGTALIKKYPKLESEFVYGDYKVYDVRKMIAKSEQEIGKATAKYFFYSNIMNFFKTEITLANGEIRKRPLIETNGETGEIVWDKGRDFATVRKVLSMPQVNIVKKTEVQTGGFSKESILPKRNSDKLIARKKDWDPKKYGGFDSPTVAYSVLVVAKVEKGKSKKLKSVKELLGITIMERSSFEKNPIDFLEAKGYKEVKKDLIIKLPKYSLFELENGRKRMLASAGELQKGNELALPSKYVNFLYLASHYEKLKGSPEDNEQKQLFVEQHKHYLDEIIEQISEFSKRVILADANLDKVLSAYNKHRDKPIREQAENIIHLFTLTNLGAPAAFKYFDTTIDRKRYTSTKEVLDATLIHQSITGLYETRIDLSQLGGDKRPAATKKAGQAKKKKAS

SEQ ID NO: 52 - DNA, 4830 bp, artificial sequence
  DNA sequence encoding artificial protein C4C9v1
atgggtgatcattatctggatattcggctgaggcctgatccagagttcccacctgcgcagctgatgtctgtcctttttggcaaacttcatcaggccctggttgcccagggcggagatcggataggggtaagctttccagacctcgacgaaagccggagccgcctgggagaacgcctgcggatccacgcttctgccgacgatctgagagccttgctggcaaggccatggcttgaggggctccgggatcacctgcagtttggcgaacccgccgttgttccccacccaaccccttatcggcaggtgtctagagtgcaggccaaatctaatccagaacggctgcgacggcgactcatgcggcgacatgatcttagcgaggaagaggcccgaaaaagaatccctgataccgtggcccgcgcccttgacttgccttttgtcacactgcggtcccagagtacggggcagcatttcagacttttcattcgacacgggccactgcaagttaccgccgaagaaggaggctttacttgttatggactctccaagggaggtttcgtgccctggtttttcgaaggcggaggcggaagtggtggcggaggatctggcggcggaggatccgctaggatggccccaaagaagaagcggaaggtcggtatccacggagtcccagcagccgacaagaagtacagcatcggcctggacatcggcaccaactctgtgggctgggccgtgatcaccgacgagtacaaggtgcccagcaagaaattcaaggtgctgggcaacaccgaccggcacagcatcaagaagaacctgatcggagccctgctgttcgacagcggcgaaacagccgaggccacccggctgaagagaaccgccagaagaagatacaccagacggaagaaccggatctgctatctgcaagagatcttcagcaacgagatggccaaggtggacgacagcttcttccacagactggaagagtccttcctggtggaagaggataagaagcacgagcggcaccccatcttcggcaacatcgtggacgaggtggcctaccacgagaagtaccccaccatctaccacctgagaaagaaactggtggacagcaccgacaaggccgacctgcggctgatctatctggccctggcccacatgatcaagttccggggccacttcctgatcgagggcgacctgaaccccgacaacagcgacgtggacaagctgttcatccagctggtgcagacctacaaccagctgttcgaggaaaaccccatcaacgccagcggcgtggacgccaaggccatcctgtctgccagactgagcaagagcagacggctggaaaatctgatcgcccagctgcccggcgagaagaagaatggcctgttcggaaacctgattgccctgagcctgggcctgacccccaacttcaagagcaacttcgacctggccgaggatgccaaactgcagctgagcaaggacacctacgacgacgacctggacaacctgctggcccagatcggcgaccagtacgccgacctgtttctggccgccaagaacctgtccgacgccatcctgctgagcgacatcctgagagtgaacaccgagatcaccaaggcccccctgagcgcctctatgatcaagagatacgacgagcaccaccaggacctgaccctgctgaaagctctcgtgcggcagcagctgcctgagaagtacaaagagattttcttcgaccagagcaagaacggctacgccggctacattgacggcggagccagccaggaagagttctacaagttcatcaagcccatcctggaaaagatggacggcaccgaggaactgctcgtgaagctgaacagagaggacctgctgcggaagcagcggaccttcgacaacggcagcatcccccaccagatccacctgggagagctgcacgccattctgcggcggcaggaagatttttacccattcctgaaggacaaccgggaaaagatcgagaagatcctgaccttccgcatcccctactacgtgggccctctggccaggggaaacagcagattcgcctggatgaccagaaagagcgaggaaaccatcaccccctggaacttcgaggaagtggtggacaagggcgcttccgcccagagcttcatcgagcggatgaccaacttcgataagaacctgcccaacgagaaggtgctgcccaagcacagcctgctgtacgagtacttcaccgtgtataacgagctgaccaaagtgaaatacgtgaccgagggaatgagaaagcccgccttcctgagcggcgagcagaaaaaggccatcgtggacctgctgttcaagaccaaccggaaagtgaccgtgaagcagctgaaagaggactacttcaagaaaatcgagtgcttcgactccgtggaaatctccggcgtggaagatcggttcaacgcctccctgggcacataccacgatctgctgaaaattatcaaggacaaggacttcctggacaatgaggaaaacgaggacattctggaagatatcgtgctgaccctgacactgtttgaggacagagagatgatcgaggaacggctgaaaacctatgcccacctgttcgacgacaaagtgatgaagcagctgaagcggcggagatacaccggctggggcaggctgagccggaagctgatcaacggcatccgggacaagcagtccggcaagacaatcctggatttcctgaagtccgacggcttcgccaacagaaacttcatgcagctgatccacgacgacagcctgacctttaaagaggacatccagaaagcccaggtgtccggccagggcgatagcctgcacgagcacattgccaatctggccggcagccccgccattaagaagggcatcctgcagacagtgaaggtggtggacgagctcgtgaaagtgatgggccggcacaagcccgagaacatcgtgatcgaaatggccagagagaaccagaccacccagaagggacagaagaacagccgcgagagaatgaagcggatcgaagagggcatcaaagagctgggcagccagatcctgaaagaacaccccgtggaaaacacccagctgcagaacgagaagctgtacctgtactacctgcagaatgggcgggatatgtacgtggaccaggaactggacatcaaccggctgtccgactacgatgtggaccatatcgtgcctcagagctttctgaaggacgactccatcgacaacaaggtgctgaccagaagcgacaagaaccggggcaagagcgacaacgtgccctccgaagaggtcgtgaagaagatgaagaactactggcggcagctgctgaacgccaagctgattacccagagaaagttcgacaatctgaccaaggccgagagaggcggcctgagcgaactggataaggccggcttcatcaagagacagctggtggaaacccggcagatcacaaagcacgtggcacagatcctggactcccggatgaacactaagtacgacgagaatgacaagctgatccgggaagtgaaagtgatcaccctgaagtccaagctggtgtccgatttccggaaggatttccagttttacaaagtgcgcgagatcaacaactaccaccacgcccacgacgcctacctgaacgccgtcgtgggaaccgccctgatcaaaaagtaccctaagctggaaagcgagttcgtgtacggcgactacaaggtgtacgacgtgcggaagatgatcgccaagagcgagcaggaaatcggcaaggctaccgccaagtacttcttctacagcaacatcatgaactttttcaagaccgagattaccctggccaacggcgagatccggaagcggcctctgatcgagacaaacggcgaaaccggggagatcgtgtgggataagggccgggattttgccaccgtgcggaaagtgctgagcatgccccaagtgaatatcgtgaaaaagaccgaggtgcagacaggcggcttcagcaaagagtctatcctgcccaagaggaacagcgataagctgatcgccagaaagaaggactgggaccctaagaagtacggcggcttcgacagccccaccgtggcctattctgtgctggtggtggccaaagtggaaaagggcaagtccaagaaactgaagagtgtgaaagagctgctggggatcaccatcatggaaagaagcagcttcgagaagaatcccatcgactttctggaagccaagggctacaaagaagtgaaaaaggacctgatcatcaagctgcctaagtactccctgttcgagctggaaaacggccggaagagaatgctggcctctgccggcgaactgcagaagggaaacgaactggccctgccctccaaatatgtgaacttcctgtacctggccagccactatgagaagctgaagggctcccccgaggataatgagcagaaacagctgtttgtggaacagcacaagcactacctggacgagatcatcgagcagatcagcgagttctccaagagagtgatcctggccgacgctaatctggacaaagtgctgtccgcctacaacaagcaccgggataagcccatcagagagcaggccgagaatatcatccacctgtttaccctgaccaatctgggagcccctgccgccttcaagtactttgacaccaccatcgaccggaagaggtacaccagcaccaaagaggtgctggacgccaccctgatccaccagagcatcaccggcctgtacgagacacggatcgacctgtctcagctgggaggcgacaagcgtcctgctgctactaagaaagctggtcaagctaagaaaaagaaagctagctga

SEQ ID NO: 53 - protein, 1622 aa, artificial sequence
  artificial protein C9C4v1
MDYKDDDDKMAPKKKRKVGIHGVPAADKKYSIGLDIGTNSVGWAVITDEYKVPSKKFKVLGNTDRHSIKKNLIGALLFDSGETAEATRLKRTARRRYTRRKNRICYLQEIFSNEMAKVDDSFFHRLEESFLVEEDKKHERHPIFGNIVDEVAYHEKYPTIYHLRKKLVDSTDKADLRLIYLALAHMIKFRGHFLIEGDLNPDNSDVDKLFIQLVQTYNQLFEENPINASGVDAKAILSARLSKSRRLENLIAQLPGEKKNGLFGNLIALSLGLTPNFKSNFDLAEDAKLQLSKDTYDDDLDNLLAQIGDQYADLFLAAKNLSDAILLSDILRVNTEITKAPLSASMIKRYDEHHQDLTLLKALVRQQLPEKYKEIFFDQSKNGYAGYIDGGASQEEFYKFIKPILEKMDGTEELLVKLNREDLLRKQRTFDNGSIPHQIHLGELHAILRRQEDFYPFLKDNREKIEKILTFRIPYYVGPLARGNSRFAWMTRKSEETITPWNFEEVVDKGASAQSFIERMTNFDKNLPNEKVLPKHSLLYEYFTVYNELTKVKYVTEGMRKPAFLSGEQKKAIVDLLFKTNRKVTVKQLKEDYFKKIECFDSVEISGVEDRFNASLGTYHDLLKIIKDKDFLDNEENEDILEDIVLTLTLFEDREMIEERLKTYAHLFDDKVMKQLKRRRYTGWGRLSRKLINGIRDKQSGKTILDFLKSDGFANRNFMQLIHDDSLTFKEDIQKAQVSGQGDSLHEHIANLAGSPAIKKGILQTVKVVDELVKVMGRHKPENIVIEMARENQTTQKGQKNSRERMKRIEEGIKELGSQILKEHPVENTQLQNEKLYLYYLQNGRDMYVDQELDINRLSDYDVDHIVPQSFLKDDSIDNKVLTRSDKNRGKSDNVPSEEVVKKMKNYWRQLLNAKLITQRKFDNLTKAERGGLSELDKAGFIKRQLVETRQITKHVAQILDSRMNTKYDENDKLIREVKVITLKSKLVSDFRKDFQFYKVREINNYHHAHDAYLNAVVGTALIKKYPKLESEFVYGDYKVYDVRKMIAKSEQEIGKATAKYFFYSNIMNFFKTEITLANGEIRKRPLIETNGETGEIVWDKGRDFATVRKVLSMPQVNIVKKTEVQTGGFSKESILPKRNSDKLIARKKDWDPKKYGGFDSPTVAYSVLVVAKVEKGKSKKLKSVKELLGITIMERSSFEKNPIDFLEAKGYKEVKKDLIIKLPKYSLFELENGRKRMLASAGELQKGNELALPSKYVNFLYLASHYEKLKGSPEDNEQKQLFVEQHKHYLDEIIEQISEFSKRVILADANLDKVLSAYNKHRDKPIREQAENIIHLFTLTNLGAPAAFKYFDTTIDRKRYTSTKEVLDATLIHQSITGLYETRIDLSQLGGDKRPAATKKAGQAKKKKASGSGLQFEGGGGSGGGGSGGGGSASGDHYLDIRLRPDPEFPPAQLMSVLFGKLHQALVAQGGDRIGVSFPDLDESRSRLGERLRIHASADDLRALLARPWLEGLRDHLQFGEPAVVPHPTPYRQVSRVQAKSNPERLRRRLMRRHDLSEEEARKRIPDTVARALDLPFVTLRSQSTGQHFRLFIRHGPLQVTAEEGGFTCYGLSKGGFVPWF

SEQ ID NO: 54 - DNA, 4866 bp, artificial sequence
  DNA sequence encoding artificial protein C9C4v1
atggattacaaagacgatgacgataagatggccccaaagaagaagcggaaggtcggtatccacggagtcccagcagccgacaagaagtacagcatcggcctggacatcggcaccaactctgtgggctgggccgtgatcaccgacgagtacaaggtgcccagcaagaaattcaaggtgctgggcaacaccgaccggcacagcatcaagaagaacctgatcggagccctgctgttcgacagcggcgaaacagccgaggccacccggctgaagagaaccgccagaagaagatacaccagacggaagaaccggatctgctatctgcaagagatcttcagcaacgagatggccaaggtggacgacagcttcttccacagactggaagagtccttcctggtggaagaggataagaagcacgagcggcaccccatcttcggcaacatcgtggacgaggtggcctaccacgagaagtaccccaccatctaccacctgagaaagaaactggtggacagcaccgacaaggccgacctgcggctgatctatctggccctggcccacatgatcaagttccggggccacttcctgatcgagggcgacctgaaccccgacaacagcgacgtggacaagctgttcatccagctggtgcagacctacaaccagctgttcgaggaaaaccccatcaacgccagcggcgtggacgccaaggccatcctgtctgccagactgagcaagagcagacggctggaaaatctgatcgcccagctgcccggcgagaagaagaatggcctgttcggaaacctgattgccctgagcctgggcctgacccccaacttcaagagcaacttcgacctggccgaggatgccaaactgcagctgagcaaggacacctacgacgacgacctggacaacctgctggcccagatcggcgaccagtacgccgacctgtttctggccgccaagaacctgtccgacgccatcctgctgagcgacatcctgagagtgaacaccgagatcaccaaggcccccctgagcgcctctatgatcaagagatacgacgagcaccaccaggacctgaccctgctgaaagctctcgtgcggcagcagctgcctgagaagtacaaagagattttcttcgaccagagcaagaacggctacgccggctacattgacggcggagccagccaggaagagttctacaagttcatcaagcccatcctggaaaagatggacggcaccgaggaactgctcgtgaagctgaacagagaggacctgctgcggaagcagcggaccttcgacaacggcagcatcccccaccagatccacctgggagagctgcacgccattctgcggcggcaggaagatttttacccattcctgaaggacaaccgggaaaagatcgagaagatcctgaccttccgcatcccctactacgtgggccctctggccaggggaaacagcagattcgcctggatgaccagaaagagcgaggaaaccatcaccccctggaacttcgaggaagtggtggacaagggcgcttccgcccagagcttcatcgagcggatgaccaacttcgataagaacctgcccaacgagaaggtgctgcccaagcacagcctgctgtacgagtacttcaccgtgtataacgagctgaccaaagtgaaatacgtgaccgagggaatgagaaagcccgccttcctgagcggcgagcagaaaaaggccatcgtggacctgctgttcaagaccaaccggaaagtgaccgtgaagcagctgaaagaggactacttcaagaaaatcgagtgcttcgactccgtggaaatctccggcgtggaagatcggttcaacgcctccctgggcacataccacgatctgctgaaaattatcaaggacaaggacttcctggacaatgaggaaaacgaggacattctggaagatatcgtgctgaccctgacactgtttgaggacagagagatgatcgaggaacggctgaaaacctatgcccacctgttcgacgacaaagtgatgaagcagctgaagcggcggagatacaccggctggggcaggctgagccggaagctgatcaacggcatccgggacaagcagtccggcaagacaatcctggatttcctgaagtccgacggcttcgccaacagaaacttcatgcagctgatccacgacgacagcctgacctttaaagaggacatccagaaagcccaggtgtccggccagggcgatagcctgcacgagcacattgccaatctggccggcagccccgccattaagaagggcatcctgcagacagtgaaggtggtggacgagctcgtgaaagtgatgggccggcacaagcccgagaacatcgtgatcgaaatggccagagagaaccagaccacccagaagggacagaagaacagccgcgagagaatgaagcggatcgaagagggcatcaaagagctgggcagccagatcctgaaagaacaccccgtggaaaacacccagctgcagaacgagaagctgtacctgtactacctgcagaatgggcgggatatgtacgtggaccaggaactggacatcaaccggctgtccgactacgatgtggaccatatcgtgcctcagagctttctgaaggacgactccatcgacaacaaggtgctgaccagaagcgacaagaaccggggcaagagcgacaacgtgccctccgaagaggtcgtgaagaagatgaagaactactggcggcagctgctgaacgccaagctgattacccagagaaagttcgacaatctgaccaaggccgagagaggcggcctgagcgaactggataaggccggcttcatcaagagacagctggtggaaacccggcagatcacaaagcacgtggcacagatcctggactcccggatgaacactaagtacgacgagaatgacaagctgatccgggaagtgaaagtgatcaccctgaagtccaagctggtgtccgatttccggaaggatttccagttttacaaagtgcgcgagatcaacaactaccaccacgcccacgacgcctacctgaacgccgtcgtgggaaccgccctgatcaaaaagtaccctaagctggaaagcgagttcgtgtacggcgactacaaggtgtacgacgtgcggaagatgatcgccaagagcgagcaggaaatcggcaaggctaccgccaagtacttcttctacagcaacatcatgaactttttcaagaccgagattaccctggccaacggcgagatccggaagcggcctctgatcgagacaaacggcgaaaccggggagatcgtgtgggataagggccgggattttgccaccgtgcggaaagtgctgagcatgccccaagtgaatatcgtgaaaaagaccgaggtgcagacaggcggcttcagcaaagagtctatcctgcccaagaggaacagcgataagctgatcgccagaaagaaggactgggaccctaagaagtacggcggcttcgacagccccaccgtggcctattctgtgctggtggtggccaaagtggaaaagggcaagtccaagaaactgaagagtgtgaaagagctgctggggatcaccatcatggaaagaagcagcttcgagaagaatcccatcgactttctggaagccaagggctacaaagaagtgaaaaaggacctgatcatcaagctgcctaagtactccctgttcgagctggaaaacggccggaagagaatgctggcctctgccggcgaactgcagaagggaaacgaactggccctgccctccaaatatgtgaacttcctgtacctggccagccactatgagaagctgaagggctcccccgaggataatgagcagaaacagctgtttgtggaacagcacaagcactacctggacgagatcatcgagcagatcagcgagttctccaagagagtgatcctggccgacgctaatctggacaaagtgctgtccgcctacaacaagcaccgggataagcccatcagagagcaggccgagaatatcatccacctgtttaccctgaccaatctgggagcccctgccgccttcaagtactttgacaccaccatcgaccggaagaggtacaccagcaccaaagaggtgctggacgccaccctgatccaccagagcatcaccggcctgtacgagacacggatcgacctgtctcagctgggaggcgacaagcgtcctgctgctactaagaaagctggtcaagctaagaaaaagaaagctagcggcagcggcctgcagttcgaaggcggaggcggaagtggtggcggaggatctggcggcggaggatccgctagtggtgatcattatctggatattcggctgaggcctgatccagagttcccacctgcgcagctgatgtctgtcctttttggcaaacttcatcaggccctggttgcccagggcggagatcggataggggtaagctttccagacctcgacgaaagccggagccgcctgggagaacgcctgcggatccacgcttctgccgacgatctgagagccttgctggcaaggccatggcttgaggggctccgggatcacctgcagtttggcgaacccgccgttgttccccacccaaccccttatcggcaggtgtctagagtgcaggccaaatctaatccagaacggctgcgacggcgactcatgcggcgacatgatcttagcgaggaagaggcccgaaaaagaatccctgataccgtggcccgcgcccttgacttgccttttgtcacactgcggtcccagagtacggggcagcatttcagacttttcattcgacacgggccactgcaagttaccgccgaagaaggaggctttacttgttatggactctccaagggaggtttcgtgccctggttt

SEQ ID NO: 55 - protein, 1647 aa, artificial sequence
  artificial protein C4C9v2
MVKRTADGSEFESPKKKRKVGSDYKDDDDKSALEAGGDHYLDIRLRPDPEFPPAQLMSVLFGKLHQALVAQGGDRIGVSFPDLDESRSRLGERLRLHASADDLRALLARPWLEGLRDHLQFGEPAVVPHPTPYRQVSRVQAKSNPERLRRRLMRRHDLSEEEARKRIPDTVARALDLPFVTLRSQSTGQHFRLFIRHGPLQVTAEEGGFTCYGLSKGGFVPWFFEGGGGSGGGGSGGGGSGGGGSGGGGSGGGGSGGGGSGTDKKYSIGLDIGTNSVGWAVITDEYKVPSKKFKVLGNTDRHSIKKNLIGALLFDSGETAEATRLKRTARRRYTRRKNRICYLQEIFSNEMAKVDDSFFHRLEESFLVEEDKKHERHPIFGNIVDEVAYHEKYPTIYHLRKKLVDSTDKADLRLIYLALAHMIKFRGHFLIEGDLNPDNSDVDKLFIQLVQTYNQLFEENPINASGVDAKAILSARLSKSRRLENLIAQLPGEKKNGLFGNLIALSLGLTPNFKSNFDLAEDAKLQLSKDTYDDDLDNLLAQIGDQYADLFLAAKNLSDAILLSDILRVNTEITKAPLSASMIKRYDEHHQDLTLLKALVRQQLPEKYKEIFFDQSKNGYAGYIDGGASQEEFYKFIKPILEKMDGTEELLVKLNREDLLRKQRTFDNGSIPHQIHLGELHAILRRQEDFYPFLKDNREKIEKILTFRIPYYVGPLARGNSRFAWMTRKSEETITPWNFEEVVDKGASAQSFIERMTNFDKNLPNEKVLPKHSLLYEYFTVYNELTKVKYVTEGMRKPAFLSGEQKKAIVDLLFKTNRKVTVKQLKEDYFKKIECFDSVEISGVEDRFNASLGTYHDLLKIIKDKDFLDNEENEDILEDIVLTLTLFEDREMIEERLKTYAHLFDDKVMKQLKRRRYTGWGRLSRKLINGIRDKQSGKTILDFLKSDGFANRNFMQLIHDDSLTFKEDIQKAQVSGQGDSLHEHIANLAGSPAIKKGILQTVKVVDELVKVMGRHKPENIVIEMARENQTTQKGQKNSRERMKRIEEGIKELGSQILKEHPVENTQLQNEKLYLYYLQNGRDMYVDQELDINRLSDYDVDHIVPQSFLKDDSIDNKVLTRSDKNRGKSDNVPSEEVVKKMKNYWRQLLNAKLITQRKFDNLTKAERGGLSELDKAGFIKRQLVETRQITKHVAQILDSRMNTKYDENDKLIREVKVITLKSKLVSDFRKDFQFYKVREINNYHHAHDAYLNAVVGTALIKKYPKLESEFVYGDYKVYDVRKMIAKSEQEIGKATAKYFFYSNIMNFFKTEITLANGEIRKRPLIETNGETGEIVWDKGRDFATVRKVLSMPQVNIVKKTEVQTGGFSKESILPKRNSDKLIARKKDWDPKKYGGFDSPTVAYSVLVVAKVEKGKSKKLKSVKELLGITIMERSSFEKNPIDFLEAKGYKEVKKDLIIKLPKYSLFELENGRKRMLASAGELQKGNELALPSKYVNFLYLASHYEKLKGSPEDNEQKQLFVEQHKHYLDEIIEQISEFSKRVILADANLDKVLSAYNKHRDKPIREQAENIIHLFTLTNLGAPAAFKYFDTTIDRKRYTSTKEVLDATLIHQSITGLYETRIDLSQLGGDKRPAATKKAGQAKKKKAS

SEQ ID NO: 56 - DNA, 4944 bp, artificial sequence
  DNA sequence encoding artificial protein C4C9v2
atggttaagagaacagccgatggcagcgagttcgagagccccaagaaaaagcggaaagtgggcagcgactacaaggacgacgacgacaaaagcgctctcgaggccggcggtgaccactacctggatattagactgcggcccgatcctgagttccctccagctcagctgatgagcgtgctgttcggcaaactgcatcaggccctggttgcccaaggcggcgatagaatcggagtgtcattccccgacctggacgagagcagatctagactgggcgagagactgagactgcacgcctctgccgatgatctgagagccctgcttgccagaccttggctggaaggcctgagagatcatctgcagtttggcgagcctgccgtggtgcctcatcctacaccttaccggcaggtttccagagtgcaggccaagagcaaccccgagagacttcggagaaggctgatgcggagacacgacctgtctgaggaagaggcccggaagagaatccccgacacagtggctagagccctggacctgcctttcgtgacactgagaagccagagcaccggccagcacttccggctgtttatcagacacggccctctgcaagtgaccgccgaagaaggcggctttacctgttacggcctgagcaaaggcggattcgtgccctggtttttcgaaggcggcggaggatctggcggaggtggaagcggtggtggtggatccggtggcggaggaagcggaggcggaggtagtggtggtggcggttctggcggaggcggatccggtaccgacaagaagtacagcatcggcctggacatcggcaccaactctgtgggctgggccgtgatcaccgacgagtacaaggtgcccagcaagaaattcaaggtgctgggcaacaccgaccggcacagcatcaagaagaacctgatcggagccctgctgttcgacagcggcgaaacagccgaggccacccggctgaagagaaccgccagaagaagatacaccagacggaagaaccggatctgctatctgcaagagatcttcagcaacgagatggccaaggtggacgacagcttcttccacagactggaagagtccttcctggtggaagaggataagaagcacgagcggcaccccatcttcggcaacatcgtggacgaggtggcctaccacgagaagtaccccaccatctaccacctgagaaagaaactggtggacagcaccgacaaggccgacctgcggctgatctatctggccctggcccacatgatcaagttccggggccacttcctgatcgagggcgacctgaaccccgacaacagcgacgtggacaagctgttcatccagctggtgcagacctacaaccagctgttcgaggaaaaccccatcaacgccagcggcgtggacgccaaggccatcctgtctgccagactgagcaagagcagacggctggaaaatctgatcgcccagctgcccggcgagaagaagaatggcctgttcggaaacctgattgccctgagcctgggcctgacccccaacttcaagagcaacttcgacctggccgaggatgccaaactgcagctgagcaaggacacctacgacgacgacctggacaacctgctggcccagatcggcgaccagtacgccgacctgtttctggccgccaagaacctgtccgacgccatcctgctgagcgacatcctgagagtgaacaccgagatcaccaaggcccccctgagcgcctctatgatcaagagatacgacgagcaccaccaggacctgaccctgctgaaagctctcgtgcggcagcagctgcctgagaagtacaaagagattttcttcgaccagagcaagaacggctacgccggctacattgacggcggagccagccaggaagagttctacaagttcatcaagcccatcctggaaaagatggacggcaccgaggaactgctcgtgaagctgaacagagaggacctgctgcggaagcagcggaccttcgacaacggcagcatcccccaccagatccacctgggagagctgcacgccattctgcggcggcaggaagatttttacccattcctgaaggacaaccgggaaaagatcgagaagatcctgaccttccgcatcccctactacgtgggccctctggccaggggaaacagcagattcgcctggatgaccagaaagagcgaggaaaccatcaccccctggaacttcgaggaagtggtggacaagggcgcttccgcccagagcttcatcgagcggatgaccaacttcgataagaacctgcccaacgagaaggtgctgcccaagcacagcctgctgtacgagtacttcaccgtgtataacgagctgaccaaagtgaaatacgtgaccgagggaatgagaaagcccgccttcctgagcggcgagcagaaaaaggccatcgtggacctgctgttcaagaccaaccggaaagtgaccgtgaagcagctgaaagaggactacttcaagaaaatcgagtgcttcgactccgtggaaatctccggcgtggaagatcggttcaacgcctccctgggcacataccacgatctgctgaaaattatcaaggacaaggacttcctggacaatgaggaaaacgaggacattctggaagatatcgtgctgaccctgacactgtttgaggacagagagatgatcgaggaacggctgaaaacctatgcccacctgttcgacgacaaagtgatgaagcagctgaagcggcggagatacaccggctggggcaggctgagccggaagctgatcaacggcatccgggacaagcagtccggcaagacaatcctggatttcctgaagtccgacggcttcgccaacagaaacttcatgcagctgatccacgacgacagcctgacctttaaagaggacatccagaaagcccaggtgtccggccagggcgatagcctgcacgagcacattgccaatctggccggcagccccgccattaagaagggcatcctgcagacagtgaaggtggtggacgagctcgtgaaagtgatgggccggcacaagcccgagaacatcgtgatcgaaatggccagagagaaccagaccacccagaagggacagaagaacagccgcgagagaatgaagcggatcgaagagggcatcaaagagctgggcagccagatcctgaaagaacaccccgtggaaaacacccagctgcagaacgagaagctgtacctgtactacctgcagaatgggcgggatatgtacgtggaccaggaactggacatcaaccggctgtccgactacgatgtggaccatatcgtgcctcagagctttctgaaggacgactccatcgacaacaaggtgctgaccagaagcgacaagaaccggggcaagagcgacaacgtgccctccgaagaggtcgtgaagaagatgaagaactactggcggcagctgctgaacgccaagctgattacccagagaaagttcgacaatctgaccaaggccgagagaggcggcctgagcgaactggataaggccggcttcatcaagagacagctggtggaaacccggcagatcacaaagcacgtggcacagatcctggactcccggatgaacactaagtacgacgagaatgacaagctgatccgggaagtgaaagtgatcaccctgaagtccaagctggtgtccgatttccggaaggatttccagttttacaaagtgcgcgagatcaacaactaccaccacgcccacgacgcctacctgaacgccgtcgtgggaaccgccctgatcaaaaagtaccctaagctggaaagcgagttcgtgtacggcgactacaaggtgtacgacgtgcggaagatgatcgccaagagcgagcaggaaatcggcaaggctaccgccaagtacttcttctacagcaacatcatgaactttttcaagaccgagattaccctggccaacggcgagatccggaagcggcctctgatcgagacaaacggcgaaaccggggagatcgtgtgggataagggccgggattttgccaccgtgcggaaagtgctgagcatgccccaagtgaatatcgtgaaaaagaccgaggtgcagacaggcggcttcagcaaagagtctatcctgcccaagaggaacagcgataagctgatcgccagaaagaaggactgggaccctaagaagtacggcggcttcgacagccccaccgtggcctattctgtgctggtggtggccaaagtggaaaagggcaagtccaagaaactgaagagtgtgaaagagctgctggggatcaccatcatggaaagaagcagcttcgagaagaatcccatcgactttctggaagccaagggctacaaagaagtgaaaaaggacctgatcatcaagctgcctaagtactccctgttcgagctggaaaacggccggaagagaatgctggcctctgccggcgaactgcagaagggaaacgaactggccctgccctccaaatatgtgaacttcctgtacctggccagccactatgagaagctgaagggctcccccgaggataatgagcagaaacagctgtttgtggaacagcacaagcactacctggacgagatcatcgagcagatcagcgagttctccaagagagtgatcctggccgacgctaatctggacaaagtgctgtccgcctacaacaagcaccgggataagcccatcagagagcaggccgagaatatcatccacctgtttaccctgaccaatctgggagcccctgccgccttcaagtactttgacaccaccatcgaccggaagaggtacaccagcaccaaagaggtgctggacgccaccctgatccaccagagcatcaccggcctgtacgagacacggatcgacctgtctcagctgggaggcgacaagcgtcctgctgctactaagaaagctggtcaagctaagaaaaagaaagctagctga

SEQ ID NO: 57 - protein, 1627 aa, artificial sequence
  artificial protein C4C9v3
MVKRTADGSEFESPKKKRKVGSDYKDDDDKSALEAGGDHYLDIRLRPDPEFPPAQLMSVLFGKLHQALVAQGGDRIGVSFPDLDESRSRLGERLRLHASADDLRALLARPWLEGLRDHLQFGEPAVVPHPTPYRQVSRVQAKSNPERLRRRLMRRHDLSEEEARKRIPDTVARALDLPFVTLRSQSTGQHFRLFIRHGPLQVTAEEGGFTCYGLSKGGFVPWFFEGGGGSGGGGSGGGGSGTDKKYSIGLDIGTNSVGWAVITDEYKVPSKKFKVLGNTDRHSIKKNLIGALLFDSGETAEATRLKRTARRRYTRRKNRICYLQEIFSNEMAKVDDSFFHRLEESFLVEEDKKHERHPIFGNIVDEVAYHEKYPTIYHLRKKLVDSTDKADLRLIYLALAHMIKFRGHFLIEGDLNPDNSDVDKLFIQLVQTYNQLFEENPINASGVDAKAILSARLSKSRRLENLIAQLPGEKKNGLFGNLIALSLGLTPNFKSNFDLAEDAKLQLSKDTYDDDLDNLLAQIGDQYADLFLAAKNLSDAILLSDILRVNTEITKAPLSASMIKRYDEHHQDLTLLKALVRQQLPEKYKEIFFDQSKNGYAGYIDGGASQEEFYKFIKPILEKMDGTEELLVKLNREDLLRKQRTFDNGSIPHQIHLGELHAILRRQEDFYPFLKDNREKIEKILTFRIPYYVGPLARGNSRFAWMTRKSEETITPWNFEEVVDKGASAQSFIERMTNFDKNLPNEKVLPKHSLLYEYFTVYNELTKVKYVTEGMRKPAFLSGEQKKAIVDLLFKTNRKVTVKQLKEDYFKKIECFDSVEISGVEDRFNASLGTYHDLLKIIKDKDFLDNEENEDILEDIVLTLTLFEDREMIEERLKTYAHLFDDKVMKQLKRRRYTGWGRLSRKLINGIRDKQSGKTILDFLKSDGFANRNFMQLIHDDSLTFKEDIQKAQVSGQGDSLHEHIANLAGSPAIKKGILQTVKVVDELVKVMGRHKPENIVIEMARENQTTQKGQKNSRERMKRIEEGIKELGSQILKEHPVENTQLQNEKLYLYYLQNGRDMYVDQELDINRLSDYDVDHIVPQSFLKDDSIDNKVLTRSDKNRGKSDNVPSEEVVKKMKNYWRQLLNAKLITQRKFDNLTKAERGGLSELDKAGFIKRQLVETRQITKHVAQILDSRMNTKYDENDKLIREVKVITLKSKLVSDFRKDFQFYKVREINNYHHAHDAYLNAVVGTALIKKYPKLESEFVYGDYKVYDVRKMIAKSEQEIGKATAKYFFYSNIMNFFKTEITLANGEIRKRPLIETNGETGEIVWDKGRDFATVRKVLSMPQVNIVKKTEVQTGGFSKESILPKRNSDKLIARKKDWDPKKYGGFDSPTVAYSVLVVAKVEKGKSKKLKSVKELLGITIMERSSFEKNPIDFLEAKGYKEVKKDLIIKLPKYSLFELENGRKRMLASAGELQKGNELALPSKYVNFLYLASHYEKLKGSPEDNEQKQLFVEQHKHYLDEIIEQISEFSKRVILADANLDKVLSAYNKHRDKPIREQAENIIHLFTLTNLGAPAAFKYFDTTIDRKRYTSTKEVLDATLIHQSITGLYETRIDLSQLGGDKRPAATKKAGQAKKKKAS

SEQ ID NO: 58 - DNA, 4884 bp, artificial sequence
  DNA sequence encoding artificial protein C4C9v3
atggttaagagaacagccgatggcagcgagttcgagagccccaagaaaaagcggaaagtgggcagcgactacaaggacgacgacgacaaaagcgctctcgaggccggcggtgaccactacctggatattagactgcggcccgatcctgagttccctccagctcagctgatgagcgtgctgttcggcaaactgcatcaggccctggttgcccaaggcggcgatagaatcggagtgtcattccccgacctggacgagagcagatctagactgggcgagagactgagactgcacgcctctgccgatgatctgagagccctgcttgccagaccttggctggaaggcctgagagatcatctgcagtttggcgagcctgccgtggtgcctcatcctacaccttaccggcaggtttccagagtgcaggccaagagcaaccccgagagacttcggagaaggctgatgcggagacacgacctgtctgaggaagaggcccggaagagaatccccgacacagtggctagagccctggacctgcctttcgtgacactgagaagccagagcaccggccagcacttccggctgtttatcagacacggccctctgcaagtgaccgccgaagaaggcggctttacctgttacggcctgagcaaaggcggattcgtgccctggtttttcgaaggcggcggaggatctggcggaggtggaagcggtggtggtggatccggtaccgacaagaagtacagcatcggcctggacatcggcaccaactctgtgggctgggccgtgatcaccgacgagtacaaggtgcccagcaagaaattcaaggtgctgggcaacaccgaccggcacagcatcaagaagaacctgatcggagccctgctgttcgacagcggcgaaacagccgaggccacccggctgaagagaaccgccagaagaagatacaccagacggaagaaccggatctgctatctgcaagagatcttcagcaacgagatggccaaggtggacgacagcttcttccacagactggaagagtccttcctggtggaagaggataagaagcacgagcggcaccccatcttcggcaacatcgtggacgaggtggcctaccacgagaagtaccccaccatctaccacctgagaaagaaactggtggacagcaccgacaaggccgacctgcggctgatctatctggccctggcccacatgatcaagttccggggccacttcctgatcgagggcgacctgaaccccgacaacagcgacgtggacaagctgttcatccagctggtgcagacctacaaccagctgttcgaggaaaaccccatcaacgccagcggcgtggacgccaaggccatcctgtctgccagactgagcaagagcagacggctggaaaatctgatcgcccagctgcccggcgagaagaagaatggcctgttcggaaacctgattgccctgagcctgggcctgacccccaacttcaagagcaacttcgacctggccgaggatgccaaactgcagctgagcaaggacacctacgacgacgacctggacaacctgctggcccagatcggcgaccagtacgccgacctgtttctggccgccaagaacctgtccgacgccatcctgctgagcgacatcctgagagtgaacaccgagatcaccaaggcccccctgagcgcctctatgatcaagagatacgacgagcaccaccaggacctgaccctgctgaaagctctcgtgcggcagcagctgcctgagaagtacaaagagattttcttcgaccagagcaagaacggctacgccggctacattgacggcggagccagccaggaagagttctacaagttcatcaagcccatcctggaaaagatggacggcaccgaggaactgctcgtgaagctgaacagagaggacctgctgcggaagcagcggaccttcgacaacggcagcatcccccaccagatccacctgggagagctgcacgccattctgcggcggcaggaagatttttacccattcctgaaggacaaccgggaaaagatcgagaagatcctgaccttccgcatcccctactacgtgggccctctggccaggggaaacagcagattcgcctggatgaccagaaagagcgaggaaaccatcaccccctggaacttcgaggaagtggtggacaagggcgcttccgcccagagcttcatcgagcggatgaccaacttcgataagaacctgcccaacgagaaggtgctgcccaagcacagcctgctgtacgagtacttcaccgtgtataacgagctgaccaaagtgaaatacgtgaccgagggaatgagaaagcccgccttcctgagcggcgagcagaaaaaggccatcgtggacctgctgttcaagaccaaccggaaagtgaccgtgaagcagctgaaagaggactacttcaagaaaatcgagtgcttcgactccgtggaaatctccggcgtggaagatcggttcaacgcctccctgggcacataccacgatctgctgaaaattatcaaggacaaggacttcctggacaatgaggaaaacgaggacattctggaagatatcgtgctgaccctgacactgtttgaggacagagagatgatcgaggaacggctgaaaacctatgcccacctgttcgacgacaaagtgatgaagcagctgaagcggcggagatacaccggctggggcaggctgagccggaagctgatcaacggcatccgggacaagcagtccggcaagacaatcctggatttcctgaagtccgacggcttcgccaacagaaacttcatgcagctgatccacgacgacagcctgacctttaaagaggacatccagaaagcccaggtgtccggccagggcgatagcctgcacgagcacattgccaatctggccggcagccccgccattaagaagggcatcctgcagacagtgaaggtggtggacgagctcgtgaaagtgatgggccggcacaagcccgagaacatcgtgatcgaaatggccagagagaaccagaccacccagaagggacagaagaacagccgcgagagaatgaagcggatcgaagagggcatcaaagagctgggcagccagatcctgaaagaacaccccgtggaaaacacccagctgcagaacgagaagctgtacctgtactacctgcagaatgggcgggatatgtacgtggaccaggaactggacatcaaccggctgtccgactacgatgtggaccatatcgtgcctcagagctttctgaaggacgactccatcgacaacaaggtgctgaccagaagcgacaagaaccggggcaagagcgacaacgtgccctccgaagaggtcgtgaagaagatgaagaactactggcggcagctgctgaacgccaagctgattacccagagaaagttcgacaatctgaccaaggccgagagaggcggcctgagcgaactggataaggccggcttcatcaagagacagctggtggaaacccggcagatcacaaagcacgtggcacagatcctggactcccggatgaacactaagtacgacgagaatgacaagctgatccgggaagtgaaagtgatcaccctgaagtccaagctggtgtccgatttccggaaggatttccagttttacaaagtgcgcgagatcaacaactaccaccacgcccacgacgcctacctgaacgccgtcgtgggaaccgccctgatcaaaaagtaccctaagctggaaagcgagttcgtgtacggcgactacaaggtgtacgacgtgcggaagatgatcgccaagagcgagcaggaaatcggcaaggctaccgccaagtacttcttctacagcaacatcatgaactttttcaagaccgagattaccctggccaacggcgagatccggaagcggcctctgatcgagacaaacggcgaaaccggggagatcgtgtgggataagggccgggattttgccaccgtgcggaaagtgctgagcatgccccaagtgaatatcgtgaaaaagaccgaggtgcagacaggcggcttcagcaaagagtctatcctgcccaagaggaacagcgataagctgatcgccagaaagaaggactgggaccctaagaagtacggcggcttcgacagccccaccgtggcctattctgtgctggtggtggccaaagtggaaaagggcaagtccaagaaactgaagagtgtgaaagagctgctggggatcaccatcatggaaagaagcagcttcgagaagaatcccatcgactttctggaagccaagggctacaaagaagtgaaaaaggacctgatcatcaagctgcctaagtactccctgttcgagctggaaaacggccggaagagaatgctggcctctgccggcgaactgcagaagggaaacgaactggccctgccctccaaatatgtgaacttcctgtacctggccagccactatgagaagctgaagggctcccccgaggataatgagcagaaacagctgtttgtggaacagcacaagcactacctggacgagatcatcgagcagatcagcgagttctccaagagagtgatcctggccgacgctaatctggacaaagtgctgtccgcctacaacaagcaccgggataagcccatcagagagcaggccgagaatatcatccacctgtttaccctgaccaatctgggagcccctgccgccttcaagtactttgacaccaccatcgaccggaagaggtacaccagcaccaaagaggtgctggacgccaccctgatccaccagagcatcaccggcctgtacgagacacggatcgacctgtctcagctgggaggcgacaagcgtcctgctgctactaagaaagctggtcaagctaagaaaaagaaagctagctga

SEQ ID NO: 59 - protein, 1647 aa, artificial sequence; identical to SEQ ID NO: 55
  artificial protein C4C9v2-1

SEQ ID NO: 60 - DNA, 4944 bp, artificial sequence
  DNA sequence encoding artificial protein C4C9v2-1
atggttaagagaacagccgatggcagcgagttcgagagccccaagaaaaagcggaaagtgggcagcgactacaaggacgacgacgacaaaagcgctctcgaggccggcggtgaccattatctggatattcggctgaggcctgatccagagttcccacctgcgcagctgatgtctgtcctttttggcaaacttcatcaggccctggttgcccagggcggagatcggataggggtaagctttccagacctcgacgaaagccggagccgcctgggagaacgcctgcggatccacgcttctgccgacgatctgagagccttgctggcaaggccatggcttgaggggctccgggatcacctgcagtttggcgaacccgccgttgttccccacccaaccccttatcggcaggtgtctagagtgcaggccaaatctaatccagaacggctgcgacggcgactcatgcggcgacatgatcttagcgaggaagaggcccgaaaaagaatccctgataccgtggcccgcgcccttgacttgccttttgtcacactgcggtcccagagtacggggcagcatttcagacttttcattcgacacgggccactgcaagttaccgccgaagaaggaggctttacttgttatggactctccaagggaggtttcgtgccctggtttttcgaaggcggcggaggatctggcggaggtggaagcggtggtggtggatccggtggcggaggaagcggaggcggaggtagtggtggtggcggttctggcggaggcggatccggtaccgacaagaagtacagcatcggcctggacatcggcaccaactctgtgggctgggccgtgatcaccgacgagtacaaggtgcccagcaagaaattcaaggtgctgggcaacaccgaccggcacagcatcaagaagaacctgatcggagccctgctgttcgacagcggcgaaacagccgaggccacccggctgaagagaaccgccagaagaagatacaccagacggaagaaccggatctgctatctgcaagagatcttcagcaacgagatggccaaggtggacgacagcttcttccacagactggaagagtccttcctggtggaagaggataagaagcacgagcggcaccccatcttcggcaacatcgtggacgaggtggcctaccacgagaagtaccccaccatctaccacctgagaaagaaactggtggacagcaccgacaaggccgacctgcggctgatctatctggccctggcccacatgatcaagttccggggccacttcctgatcgagggcgacctgaaccccgacaacagcgacgtggacaagctgttcatccagctggtgcagacctacaaccagctgttcgaggaaaaccccatcaacgccagcggcgtggacgccaaggccatcctgtctgccagactgagcaagagcagacggctggaaaatctgatcgcccagctgcccggcgagaagaagaatggcctgttcggaaacctgattgccctgagcctgggcctgacccccaacttcaagagcaacttcgacctggccgaggatgccaaactgcagctgagcaaggacacctacgacgacgacctggacaacctgctggcccagatcggcgaccagtacgccgacctgtttctggccgccaagaacctgtccgacgccatcctgctgagcgacatcctgagagtgaacaccgagatcaccaaggcccccctgagcgcctctatgatcaagagatacgacgagcaccaccaggacctgaccctgctgaaagctctcgtgcggcagcagctgcctgagaagtacaaagagattttcttcgaccagagcaagaacggctacgccggctacattgacggcggagccagccaggaagagttctacaagttcatcaagcccatcctggaaaagatggacggcaccgaggaactgctcgtgaagctgaacagagaggacctgctgcggaagcagcggaccttcgacaacggcagcatcccccaccagatccacctgggagagctgcacgccattctgcggcggcaggaagatttttacccattcctgaaggacaaccgggaaaagatcgagaagatcctgaccttccgcatcccctactacgtgggccctctggccaggggaaacagcagattcgcctggatgaccagaaagagcgaggaaaccatcaccccctggaacttcgaggaagtggtggacaagggcgcttccgcccagagcttcatcgagcggatgaccaacttcgataagaacctgcccaacgagaaggtgctgcccaagcacagcctgctgtacgagtacttcaccgtgtataacgagctgaccaaagtgaaatacgtgaccgagggaatgagaaagcccgccttcctgagcggcgagcagaaaaaggccatcgtggacctgctgttcaagaccaaccggaaagtgaccgtgaagcagctgaaagaggactacttcaagaaaatcgagtgcttcgactccgtggaaatctccggcgtggaagatcggttcaacgcctccctgggcacataccacgatctgctgaaaattatcaaggacaaggacttcctggacaatgaggaaaacgaggacattctggaagatatcgtgctgaccctgacactgtttgaggacagagagatgatcgaggaacggctgaaaacctatgcccacctgttcgacgacaaagtgatgaagcagctgaagcggcggagatacaccggctggggcaggctgagccggaagctgatcaacggcatccgggacaagcagtccggcaagacaatcctggatttcctgaagtccgacggcttcgccaacagaaacttcatgcagctgatccacgacgacagcctgacctttaaagaggacatccagaaagcccaggtgtccggccagggcgatagcctgcacgagcacattgccaatctggccggcagccccgccattaagaagggcatcctgcagacagtgaaggtggtggacgagctcgtgaaagtgatgggccggcacaagcccgagaacatcgtgatcgaaatggccagagagaaccagaccacccagaagggacagaagaacagccgcgagagaatgaagcggatcgaagagggcatcaaagagctgggcagccagatcctgaaagaacaccccgtggaaaacacccagctgcagaacgagaagctgtacctgtactacctgcagaatgggcgggatatgtacgtggaccaggaactggacatcaaccggctgtccgactacgatgtggaccatatcgtgcctcagagctttctgaaggacgactccatcgacaacaaggtgctgaccagaagcgacaagaaccggggcaagagcgacaacgtgccctccgaagaggtcgtgaagaagatgaagaactactggcggcagctgctgaacgccaagctgattacccagagaaagttcgacaatctgaccaaggccgagagaggcggcctgagcgaactggataaggccggcttcatcaagagacagctggtggaaacccggcagatcacaaagcacgtggcacagatcctggactcccggatgaacactaagtacgacgagaatgacaagctgatccgggaagtgaaagtgatcaccctgaagtccaagctggtgtccgatttccggaaggatttccagttttacaaagtgcgcgagatcaacaactaccaccacgcccacgacgcctacctgaacgccgtcgtgggaaccgccctgatcaaaaagtaccctaagctggaaagcgagttcgtgtacggcgactacaaggtgtacgacgtgcggaagatgatcgccaagagcgagcaggaaatcggcaaggctaccgccaagtacttcttctacagcaacatcatgaactttttcaagaccgagattaccctggccaacggcgagatccggaagcggcctctgatcgagacaaacggcgaaaccggggagatcgtgtgggataagggccgggattttgccaccgtgcggaaagtgctgagcatgccccaagtgaatatcgtgaaaaagaccgaggtgcagacaggcggcttcagcaaagagtctatcctgcccaagaggaacagcgataagctgatcgccagaaagaaggactgggaccctaagaagtacggcggcttcgacagccccaccgtggcctattctgtgctggtggtggccaaagtggaaaagggcaagtccaagaaactgaagagtgtgaaagagctgctggggatcaccatcatggaaagaagcagcttcgagaagaatcccatcgactttctggaagccaagggctacaaagaagtgaaaaaggacctgatcatcaagctgcctaagtactccctgttcgagctggaaaacggccggaagagaatgctggcctctgccggcgaactgcagaagggaaacgaactggccctgccctccaaatatgtgaacttcctgtacctggccagccactatgagaagctgaagggctcccccgaggataatgagcagaaacagctgtttgtggaacagcacaagcactacctggacgagatcatcgagcagatcagcgagttctccaagagagtgatcctggccgacgctaatctggacaaagtgctgtccgcctacaacaagcaccgggataagcccatcagagagcaggccgagaatatcatccacctgtttaccctgaccaatctgggagcccctgccgccttcaagtactttgacaccaccatcgaccggaagaggtacaccagcaccaaagaggtgctggacgccaccctgatccaccagagcatcaccggcctgtacgagacacggatcgacctgtctcagctgggaggcgacaagcgtcctgctgctactaagaaagctggtcaagctaagaaaaagaaagctagctga

SEQ ID NO: 61 - protein, 1646 aa, artificial sequence
  artificial protein C9C4v2
MDYKDDDDKMAPKKKRKVGIHGVPAADKKYSIGLDIGTNSVGWAVITDEYKVPSKKFKVLGNTDRHSIKKNLIGALLFDSGETAEATRLKRTARRRYTRRKNRICYLQEIFSNEMAKVDDSFFHRLEESFLVEEDKKHERHPIFGNIVDEVAYHEKYPTIYHLRKKLVDSTDKADLRLIYLALAHMIKFRGHFLIEGDLNPDNSDVDKLFIQLVQTYNQLFEENPINASGVDAKAILSARLSKSRRLENLIAQLPGEKKNGLFGNLIALSLGLTPNFKSNFDLAEDAKLQLSKDTYDDDLDNLLAQIGDQYADLFLAAKNLSDAILLSDILRVNTEITKAPLSASMIKRYDEHHQDLTLLKALVRQQLPEKYKEIFFDQSKNGYAGYIDGGASQEEFYKFIKPILEKMDGTEELLVKLNREDLLRKQRTFDNGSIPHQIHLGELHAILRRQEDFYPFLKDNREKIEKILTFRIPYYVGPLARGNSRFAWMTRKSEETITPWNFEEVVDKGASAQSFIERMTNFDKNLPNEKVLPKHSLLYEYFTVYNELTKVKYVTEGMRKPAFLSGEQKKAIVDLLFKTNRKVTVKQLKEDYFKKIECFDSVEISGVEDRFNASLGTYHDLLKIIKDKDFLDNEENEDILEDIVLTLTLFEDREMIEERLKTYAHLFDDKVMKQLKRRRYTGWGRLSRKLINGIRDKQSGKTILDFLKSDGFANRNFMQLIHDDSLTFKEDIQKAQVSGQGDSLHEHIANLAGSPAIKKGILQTVKVVDELVKVMGRHKPENIVIEMARENQTTQKGQKNSRERMKRIEEGIKELGSQILKEHPVENTQLQNEKLYLYYLQNGRDMYVDQELDINRLSDYDVDHIVPQSFLKDDSIDNKVLTRSDKNRGKSDNVPSEEVVKKMKNYWRQLLNAKLITQRKFDNLTKAERGGLSELDKAGFIKRQLVETRQITKHVAQILDSRMNTKYDENDKLIREVKVITLKSKLVSDFRKDFQFYKVREINNYHHAHDAYLNAVVGTALIKKYPKLESEFVYGDYKVYDVRKMIAKSEQEIGKATAKYFFYSNIMNFFKTEITLANGEIRKRPLIETNGETGEIVWDKGRDFATVRKVLSMPQVNIVKKTEVQTGGFSKESILPKRNSDKLIARKKDWDPKKYGGFDSPTVAYSVLVVAKVEKGKSKKLKSVKELLGITIMERSSFEKNPIDFLEAKGYKEVKKDLIIKLPKYSLFELENGRKRMLASAGELQKGNELALPSKYVNFLYLASHYEKLKGSPEDNEQKQLFVEQHKHYLDEIIEQISEFSKRVILADANLDKVLSAYNKHRDKPIREQAENIIHLFTLTNLGAPAAFKYFDTTIDRKRYTSTKEVLDATLIHQSITGLYETRIDLSQLGGDNCLGGGGSGGGGSGGGGSGGGGSGGGGSGGGGSGGGGSTGGDHYLDIRLRPDPEFPPAQLMSVLFGKLHQALVAQGGDRIGVSFPDLDESRSRLGERLRLHASADDLRALLARPWLEGLRDHLQFGEPAVVPHPTPYRQVSRVQAKSNPERLRRRLMRRHDLSEEEARKRIPDTVARALDLPFVTLRSQSTGQHFRLFIRHGPLQVTAEEGGFTCYGLSKGGFVPWFFESALEAGKRTADGSEFESPKKKRKV

SEQ ID NO: 62 - DNA, 4941 bp, artificial sequence
  DNA sequence encoding artificial protein C9C4v2
atggattacaaagacgatgacgataagatggccccaaagaagaagcggaaggtcggtatccacggagtcccagcagccgacaagaagtacagcatcggcctggacatcggcaccaactctgtgggctgggccgtgatcaccgacgagtacaaggtgcccagcaagaaattcaaggtgctgggcaacaccgaccggcacagcatcaagaagaacctgatcggagccctgctgttcgacagcggcgaaacagccgaggccacccggctgaagagaaccgccagaagaagatacaccagacggaagaaccggatctgctatctgcaagagatcttcagcaacgagatggccaaggtggacgacagcttcttccacagactggaagagtccttcctggtggaagaggataagaagcacgagcggcaccccatcttcggcaacatcgtggacgaggtggcctaccacgagaagtaccccaccatctaccacctgagaaagaaactggtggacagcaccgacaaggccgacctgcggctgatctatctggccctggcccacatgatcaagttccggggccacttcctgatcgagggcgacctgaaccccgacaacagcgacgtggacaagctgttcatccagctggtgcagacctacaaccagctgttcgaggaaaaccccatcaacgccagcggcgtggacgccaaggccatcctgtctgccagactgagcaagagcagacggctggaaaatctgatcgcccagctgcccggcgagaagaagaatggcctgttcggaaacctgattgccctgagcctgggcctgacccccaacttcaagagcaacttcgacctggccgaggatgccaaactgcagctgagcaaggacacctacgacgacgacctggacaacctgctggcccagatcggcgaccagtacgccgacctgtttctggccgccaagaacctgtccgacgccatcctgctgagcgacatcctgagagtgaacaccgagatcaccaaggcccccctgagcgcctctatgatcaagagatacgacgagcaccaccaggacctgaccctgctgaaagctctcgtgcggcagcagctgcctgagaagtacaaagagattttcttcgaccagagcaagaacggctacgccggctacattgacggcggagccagccaggaagagttctacaagttcatcaagcccatcctggaaaagatggacggcaccgaggaactgctcgtgaagctgaacagagaggacctgctgcggaagcagcggaccttcgacaacggcagcatcccccaccagatccacctgggagagctgcacgccattctgcggcggcaggaagatttttacccattcctgaaggacaaccgggaaaagatcgagaagatcctgaccttccgcatcccctactacgtgggccctctggccaggggaaacagcagattcgcctggatgaccagaaagagcgaggaaaccatcaccccctggaacttcgaggaagtggtggacaagggcgcttccgcccagagcttcatcgagcggatgaccaacttcgataagaacctgcccaacgagaaggtgctgcccaagcacagcctgctgtacgagtacttcaccgtgtataacgagctgaccaaagtgaaatacgtgaccgagggaatgagaaagcccgccttcctgagcggcgagcagaaaaaggccatcgtggacctgctgttcaagaccaaccggaaagtgaccgtgaagcagctgaaagaggactacttcaagaaaatcgagtgcttcgactccgtggaaatctccggcgtggaagatcggttcaacgcctccctgggcacataccacgatctgctgaaaattatcaaggacaaggacttcctggacaatgaggaaaacgaggacattctggaagatatcgtgctgaccctgacactgtttgaggacagagagatgatcgaggaacggctgaaaacctatgcccacctgttcgacgacaaagtgatgaagcagctgaagcggcggagatacaccggctggggcaggctgagccggaagctgatcaacggcatccgggacaagcagtccggcaagacaatcctggatttcctgaagtccgacggcttcgccaacagaaacttcatgcagctgatccacgacgacagcctgacctttaaagaggacatccagaaagcccaggtgtccggccagggcgatagcctgcacgagcacattgccaatctggccggcagccccgccattaagaagggcatcctgcagacagtgaaggtggtggacgagctcgtgaaagtgatgggccggcacaagcccgagaacatcgtgatcgaaatggccagagagaaccagaccacccagaagggacagaagaacagccgcgagagaatgaagcggatcgaagagggcatcaaagagctgggcagccagatcctgaaagaacaccccgtggaaaacacccagctgcagaacgagaagctgtacctgtactacctgcagaatgggcgggatatgtacgtggaccaggaactggacatcaaccggctgtccgactacgatgtggaccatatcgtgcctcagagctttctgaaggacgactccatcgacaacaaggtgctgaccagaagcgacaagaaccggggcaagagcgacaacgtgccctccgaagaggtcgtgaagaagatgaagaactactggcggcagctgctgaacgccaagctgattacccagagaaagttcgacaatctgaccaaggccgagagaggcggcctgagcgaactggataaggccggcttcatcaagagacagctggtggaaacccggcagatcacaaagcacgtggcacagatcctggactcccggatgaacactaagtacgacgagaatgacaagctgatccgggaagtgaaagtgatcaccctgaagtccaagctggtgtccgatttccggaaggatttccagttttacaaagtgcgcgagatcaacaactaccaccacgcccacgacgcctacctgaacgccgtcgtgggaaccgccctgatcaaaaagtaccctaagctggaaagcgagttcgtgtacggcgactacaaggtgtacgacgtgcggaagatgatcgccaagagcgagcaggaaatcggcaaggctaccgccaagtacttcttctacagcaacatcatgaactttttcaagaccgagattaccctggccaacggcgagatccggaagcggcctctgatcgagacaaacggcgaaaccggggagatcgtgtgggataagggccgggattttgccaccgtgcggaaagtgctgagcatgccccaagtgaatatcgtgaaaaagaccgaggtgcagacaggcggcttcagcaaagagtctatcctgcccaagaggaacagcgataagctgatcgccagaaagaaggactgggaccctaagaagtacggcggcttcgacagccccaccgtggcctattctgtgctggtggtggccaaagtggaaaagggcaagtccaagaaactgaagagtgtgaaagagctgctggggatcaccatcatggaaagaagcagcttcgagaagaatcccatcgactttctggaagccaagggctacaaagaagtgaaaaaggacctgatcatcaagctgcctaagtactccctgttcgagctggaaaacggccggaagagaatgctggcctctgccggcgaactgcagaagggaaacgaactggccctgccctccaaatatgtgaacttcctgtacctggccagccactatgagaagctgaagggctcccccgaggataatgagcagaaacagctgtttgtggaacagcacaagcactacctggacgagatcatcgagcagatcagcgagttctccaagagagtgatcctggccgacgctaatctggacaaagtgctgtccgcctacaacaagcaccgggataagcccatcagagagcaggccgagaatatcatccacctgtttaccctgaccaatctgggagcccctgccgccttcaagtactttgacaccaccatcgaccggaagaggtacaccagcaccaaagaggtgctggacgccaccctgatccaccagagcatcaccggcctgtacgagacacggatcgacctgtctcagctgggaggcgacaattgtctgggtggcggaggaagcggaggcggcggatctggcggcggaggatccggcggtggtggttctggcggtggcggtagtggcggaggtggtagcggtggtggcggatccaccggcggtgaccactacctggatattagactgcggcccgatcctgagttccctccagctcagctgatgagcgtgctgttcggcaaactgcatcaggccctggttgcccaaggcggcgatagaatcggagtgtcattccccgacctggacgagagcagatctagactgggcgagagactgagactgcacgcctctgccgatgatctgagagccctgcttgccagaccttggctggaaggcctgagagatcatctgcagtttggcgagcctgccgtggtgcctcatcctacaccttaccggcaggtttccagagtgcaggccaagagcaaccccgagagacttcggagaaggctgatgcggagacacgacctgtctgaggaagaggcccggaagagaatccccgacacagtggctagagccctggacctgcctttcgtgacactgagaagccagagcaccggccagcacttccggctgtttatcagacacggccctctgcaagtgaccgccgaagaaggcggctttacctgttacggcctgagcaaaggcggattcgtgccctggtttttcgaaagcgctctcgaggccggcaaaagaaccgccgatggcagcgagtttgagagccctaagaaaaaacggaaggtgtag

SEQ ID NO: 63 - protein, 1626 aa, artificial sequence
  artificial protein C9C4v3
MDYKDDDDKMAPKKKRKVGIHGVPAADKKYSIGLDIGTNSVGWAVITDEYKVPSKKFKVLGNTDRHSIKKNLIGALLFDSGETAEATRLKRTARRRYTRRKNRICYLQEIFSNEMAKVDDSFFHRLEESFLVEEDKKHERHPIFGNIVDEVAYHEKYPTIYHLRKKLVDSTDKADLRLIYLALAHMIKFRGHFLIEGDLNPDNSDVDKLFIQLVQTYNQLFEENPINASGVDAKAILSARLSKSRRLENLIAQLPGEKKNGLFGNLIALSLGLTPNFKSNFDLAEDAKLQLSKDTYDDDLDNLLAQIGDQYADLFLAAKNLSDAILLSDILRVNTEITKAPLSASMIKRYDEHHQDLTLLKALVRQQLPEKYKEIFFDQSKNGYAGYIDGGASQEEFYKFIKPILEKMDGTEELLVKLNREDLLRKQRTFDNGSIPHQIHLGELHAILRRQEDFYPFLKDNREKIEKILTFRIPYYVGPLARGNSRFAWMTRKSEETITPWNFEEVVDKGASAQSFIERMTNFDKNLPNEKVLPKHSLLYEYFTVYNELTKVKYVTEGMRKPAFLSGEQKKAIVDLLFKTNRKVTVKQLKEDYFKKIECFDSVEISGVEDRFNASLGTYHDLLKIIKDKDFLDNEENEDILEDIVLTLTLFEDREMIEERLKTYAHLFDDKVMKQLKRRRYTGWGRLSRKLINGIRDKQSGKTILDFLKSDGFANRNFMQLIHDDSLTFKEDIQKAQVSGQGDSLHEHIANLAGSPAIKKGILQTVKVVDELVKVMGRHKPENIVIEMARENQTTQKGQKNSRERMKRIEEGIKELGSQILKEHPVENTQLQNEKLYLYYLQNGRDMYVDQELDINRLSDYDVDHIVPQSFLKDDSIDNKVLTRSDKNRGKSDNVPSEEVVKKMKNYWRQLLNAKLITQRKFDNLTKAERGGLSELDKAGFIKRQLVETRQITKHVAQILDSRMNTKYDENDKLIREVKVITLKSKLVSDFRKDFQFYKVREINNYHHAHDAYLNAVVGTALIKKYPKLESEFVYGDYKVYDVRKMIAKSEQEIGKATAKYFFYSNIMNFFKTEITLANGEIRKRPLIETNGETGEIVWDKGRDFATVRKVLSMPQVNIVKKTEVQTGGFSKESILPKRNSDKLIARKKDWDPKKYGGFDSPTVAYSVLVVAKVEKGKSKKLKSVKELLGITIMERSSFEKNPIDFLEAKGYKEVKKDLIIKLPKYSLFELENGRKRMLASAGELQKGNELALPSKYVNFLYLASHYEKLKGSPEDNEQKQLFVEQHKHYLDEIIEQISEFSKRVILADANLDKVLSAYNKHRDKPIREQAENIIHLFTLTNLGAPAAFKYFDTTIDRKRYTSTKEVLDATLIHQSITGLYETRIDLSQLGGDNCLGGGGSGGGGSGGGGSTGGDHYLDIRLRPDPEFPPAQLMSVLFGKLHQALVAQGGDRIGVSFPDLDESRSRLGERLRLHASADDLRALLARPWLEGLRDHLQFGEPAVVPHPTPYRQVSRVQAKSNPERLRRRLMRRHDLSEEEARKRIPDTVARALDLPFVTLRSQSTGQHFRLFIRHGPLQVTAEEGGFTCYGLSKGGFVPWFFESALEAGKRTADGSEFESPKKKRKV

SEQ ID NO: 64 - DNA, 4881 bp, artificial sequence
  DNA sequence encoding artificial protein C9C4v3
atggattacaaagacgatgacgataagatggccccaaagaagaagcggaaggtcggtatccacggagtcccagcagccgacaagaagtacagcatcggcctggacatcggcaccaactctgtgggctgggccgtgatcaccgacgagtacaaggtgcccagcaagaaattcaaggtgctgggcaacaccgaccggcacagcatcaagaagaacctgatcggagccctgctgttcgacagcggcgaaacagccgaggccacccggctgaagagaaccgccagaagaagatacaccagacggaagaaccggatctgctatctgcaagagatcttcagcaacgagatggccaaggtggacgacagcttcttccacagactggaagagtccttcctggtggaagaggataagaagcacgagcggcaccccatcttcggcaacatcgtggacgaggtggcctaccacgagaagtaccccaccatctaccacctgagaaagaaactggtggacagcaccgacaaggccgacctgcggctgatctatctggccctggcccacatgatcaagttccggggccacttcctgatcgagggcgacctgaaccccgacaacagcgacgtggacaagctgttcatccagctggtgcagacctacaaccagctgttcgaggaaaaccccatcaacgccagcggcgtggacgccaaggccatcctgtctgccagactgagcaagagcagacggctggaaaatctgatcgcccagctgcccggcgagaagaagaatggcctgttcggaaacctgattgccctgagcctgggcctgacccccaacttcaagagcaacttcgacctggccgaggatgccaaactgcagctgagcaaggacacctacgacgacgacctggacaacctgctggcccagatcggcgaccagtacgccgacctgtttctggccgccaagaacctgtccgacgccatcctgctgagcgacatcctgagagtgaacaccgagatcaccaaggcccccctgagcgcctctatgatcaagagatacgacgagcaccaccaggacctgaccctgctgaaagctctcgtgcggcagcagctgcctgagaagtacaaagagattttcttcgaccagagcaagaacggctacgccggctacattgacggcggagccagccaggaagagttctacaagttcatcaagcccatcctggaaaagatggacggcaccgaggaactgctcgtgaagctgaacagagaggacctgctgcggaagcagcggaccttcgacaacggcagcatcccccaccagatccacctgggagagctgcacgccattctgcggcggcaggaagatttttacccattcctgaaggacaaccgggaaaagatcgagaagatcctgaccttccgcatcccctactacgtgggccctctggccaggggaaacagcagattcgcctggatgaccagaaagagcgaggaaaccatcaccccctggaacttcgaggaagtggtggacaagggcgcttccgcccagagcttcatcgagcggatgaccaacttcgataagaacctgcccaacgagaaggtgctgcccaagcacagcctgctgtacgagtacttcaccgtgtataacgagctgaccaaagtgaaatacgtgaccgagggaatgagaaagcccgccttcctgagcggcgagcagaaaaaggccatcgtggacctgctgttcaagaccaaccggaaagtgaccgtgaagcagctgaaagaggactacttcaagaaaatcgagtgcttcgactccgtggaaatctccggcgtggaagatcggttcaacgcctccctgggcacataccacgatctgctgaaaattatcaaggacaaggacttcctggacaatgaggaaaacgaggacattctggaagatatcgtgctgaccctgacactgtttgaggacagagagatgatcgaggaacggctgaaaacctatgcccacctgttcgacgacaaagtgatgaagcagctgaagcggcggagatacaccggctggggcaggctgagccggaagctgatcaacggcatccgggacaagcagtccggcaagacaatcctggatttcctgaagtccgacggcttcgccaacagaaacttcatgcagctgatccacgacgacagcctgacctttaaagaggacatccagaaagcccaggtgtccggccagggcgatagcctgcacgagcacattgccaatctggccggcagccccgccattaagaagggcatcctgcagacagtgaaggtggtggacgagctcgtgaaagtgatgggccggcacaagcccgagaacatcgtgatcgaaatggccagagagaaccagaccacccagaagggacagaagaacagccgcgagagaatgaagcggatcgaagagggcatcaaagagctgggcagccagatcctgaaagaacaccccgtggaaaacacccagctgcagaacgagaagctgtacctgtactacctgcagaatgggcgggatatgtacgtggaccaggaactggacatcaaccggctgtccgactacgatgtggaccatatcgtgcctcagagctttctgaaggacgactccatcgacaacaaggtgctgaccagaagcgacaagaaccggggcaagagcgacaacgtgccctccgaagaggtcgtgaagaagatgaagaactactggcggcagctgctgaacgccaagctgattacccagagaaagttcgacaatctgaccaaggccgagagaggcggcctgagcgaactggataaggccggcttcatcaagagacagctggtggaaacccggcagatcacaaagcacgtggcacagatcctggactcccggatgaacactaagtacgacgagaatgacaagctgatccgggaagtgaaagtgatcaccctgaagtccaagctggtgtccgatttccggaaggatttccagttttacaaagtgcgcgagatcaacaactaccaccacgcccacgacgcctacctgaacgccgtcgtgggaaccgccctgatcaaaaagtaccctaagctggaaagcgagttcgtgtacggcgactacaaggtgtacgacgtgcggaagatgatcgccaagagcgagcaggaaatcggcaaggctaccgccaagtacttcttctacagcaacatcatgaactttttcaagaccgagattaccctggccaacggcgagatccggaagcggcctctgatcgagacaaacggcgaaaccggggagatcgtgtgggataagggccgggattttgccaccgtgcggaaagtgctgagcatgccccaagtgaatatcgtgaaaaagaccgaggtgcagacaggcggcttcagcaaagagtctatcctgcccaagaggaacagcgataagctgatcgccagaaagaaggactgggaccctaagaagtacggcggcttcgacagccccaccgtggcctattctgtgctggtggtggccaaagtggaaaagggcaagtccaagaaactgaagagtgtgaaagagctgctggggatcaccatcatggaaagaagcagcttcgagaagaatcccatcgactttctggaagccaagggctacaaagaagtgaaaaaggacctgatcatcaagctgcctaagtactccctgttcgagctggaaaacggccggaagagaatgctggcctctgccggcgaactgcagaagggaaacgaactggccctgccctccaaatatgtgaacttcctgtacctggccagccactatgagaagctgaagggctcccccgaggataatgagcagaaacagctgtttgtggaacagcacaagcactacctggacgagatcatcgagcagatcagcgagttctccaagagagtgatcctggccgacgctaatctggacaaagtgctgtccgcctacaacaagcaccgggataagcccatcagagagcaggccgagaatatcatccacctgtttaccctgaccaatctgggagcccctgccgccttcaagtactttgacaccaccatcgaccggaagaggtacaccagcaccaaagaggtgctggacgccaccctgatccaccagagcatcaccggcctgtacgagacacggatcgacctgtctcagctgggaggcgacaattgtctgggtggcggaggaagcggaggcggcggatctggcggcggaggatccaccggcggtgaccactacctggatattagactgcggcccgatcctgagttccctccagctcagctgatgagcgtgctgttcggcaaactgcatcaggccctggttgcccaaggcggcgatagaatcggagtgtcattccccgacctggacgagagcagatctagactgggcgagagactgagactgcacgcctctgccgatgatctgagagccctgcttgccagaccttggctggaaggcctgagagatcatctgcagtttggcgagcctgccgtggtgcctcatcctacaccttaccggcaggtttccagagtgcaggccaagagcaaccccgagagacttcggagaaggctgatgcggagacacgacctgtctgaggaagaggcccggaagagaatccccgacacagtggctagagccctggacctgcctttcgtgacactgagaagccagagcaccggccagcacttccggctgtttatcagacacggccctctgcaagtgaccgccgaagaaggcggctttacctgttacggcctgagcaaaggcggattcgtgccctggtttttcgaaagcgctctcgaggccggcaaaagaaccgccgatggcagcgagtttgagagccctaagaaaaaacggaaggtgtag

SEQ ID NO: 65 - protein, 1646 aa, artificial sequence
  artificial protein C9C4v2-1
MDYKDDDDKMAPKKKRKVGIHGVPAADKKYSIGLDIGTNSVGWAVITDEYKVPSKKFKVLGNTDRHSIKKNLIGALLFDSGETAEATRLKRTARRRYTRRKNRICYLQEIFSNEMAKVDDSFFHRLEESFLVEEDKKHERHPIFGNIVDEVAYHEKYPTIYHLRKKLVDSTDKADLRLIYLALAHMIKFRGHFLIEGDLNPDNSDVDKLFIQLVQTYNQLFEENPINASGVDAKAILSARLSKSRRLENLIAQLPGEKKNGLFGNLIALSLGLTPNFKSNFDLAEDAKLQLSKDTYDDDLDNLLAQIGDQYADLFLAAKNLSDAILLSDILRVNTEITKAPLSASMIKRYDEHHQDLTLLKALVRQQLPEKYKEIFFDQSKNGYAGYIDGGASQEEFYKFIKPILEKMDGTEELLVKLNREDLLRKQRTFDNGSIPHQIHLGELHAILRRQEDFYPFLKDNREKIEKILTFRIPYYVGPLARGNSRFAWMTRKSEETITPWNFEEVVDKGASAQSFIERMTNFDKNLPNEKVLPKHSLLYEYFTVYNELTKVKYVTEGMRKPAFLSGEQKKAIVDLLFKTNRKVTVKQLKEDYFKKIECFDSVEISGVEDRFNASLGTYHDLLKIIKDKDFLDNEENEDILEDIVLTLTLFEDREMIEERLKTYAHLFDDKVMKQLKRRRYTGWGRLSRKLINGIRDKQSGKTILDFLKSDGFANRNFMQLIHDDSLTFKEDIQKAQVSGQGDSLHEHIANLAGSPAIKKGILQTVKVVDELVKVMGRHKPENIVIEMARENQTTQKGQKNSRERMKRIEEGIKELGSQILKEHPVENTQLQNEKLYLYYLQNGRDMYVDQELDINRLSDYDVDHIVPQSFLKDDSIDNKVLTRSDKNRGKSDNVPSEEVVKKMKNYWRQLLNAKLITQRKFDNLTKAERGGLSELDKAGFIKRQLVETRQITKHVAQILDSRMNTKYDENDKLIREVKVITLKSKLVSDFRKDFQFYKVREINNYHHAHDAYLNAVVGTALIKKYPKLESEFVYGDYKVYDVRKMIAKSEQEIGKATAKYFFYSNIMNFFKTEITLANGEIRKRPLIETNGETGEIVWDKGRDFATVRKVLSMPQVNIVKKTEVQTGGFSKESILPKRNSDKLIARKKDWDPKKYGGFDSPTVAYSVLVVAKVEKGKSKKLKSVKELLGITIMERSSFEKNPIDFLEAKGYKEVKKDLIIKLPKYSLFELENGRKRMLASAGELQKGNELALPSKYVNFLYLASHYEKLKGSPEDNEQKQLFVEQHKHYLDEIIEQISEFSKRVILADANLDKVLSAYNKHRDKPIREQAENIIHLFTLTNLGAPAAFKYFDTTIDRKRYTSTKEVLDATLIHQSITGLYETRIDLSQLGGDNCLGGGGSGGGGSGGGGSGGGGSGGGGSGGGGSGGGGSTGGDHYLDIRLRPDPEFPPAQLMSVLFGKLHQALVAQGGDRIGVSFPDLDESRSRLGERLRIHASADDLRALLARPWLEGLRDHLQFGEPAVVPHPTPYRQVSRVQAKSNPERLRRRLMRRHDLSEEEARKRIPDTVARALDLPFVTLRSQSTGQHFRLFIRHGPLQVTAEEGGFTCYGLSKGGFVPWFFESALEAGKRTADGSEFESPKKKRKV

SEQ ID NO: 66 - DNA, 4941 bp, artificial sequence
  DNA sequence encoding artificial protein C9C4v2-1
atggattacaaagacgatgacgataagatggccccaaagaagaagcggaaggtcggtatccacggagtcccagcagccgacaagaagtacagcatcggcctggacatcggcaccaactctgtgggctgggccgtgatcaccgacgagtacaaggtgcccagcaagaaattcaaggtgctgggcaacaccgaccggcacagcatcaagaagaacctgatcggagccctgctgttcgacagcggcgaaacagccgaggccacccggctgaagagaaccgccagaagaagatacaccagacggaagaaccggatctgctatctgcaagagatcttcagcaacgagatggccaaggtggacgacagcttcttccacagactggaagagtccttcctggtggaagaggataagaagcacgagcggcaccccatcttcggcaacatcgtggacgaggtggcctaccacgagaagtaccccaccatctaccacctgagaaagaaactggtggacagcaccgacaaggccgacctgcggctgatctatctggccctggcccacatgatcaagttccggggccacttcctgatcgagggcgacctgaaccccgacaacagcgacgtggacaagctgttcatccagctggtgcagacctacaaccagctgttcgaggaaaaccccatcaacgccagcggcgtggacgccaaggccatcctgtctgccagactgagcaagagcagacggctggaaaatctgatcgcccagctgcccggcgagaagaagaatggcctgttcggaaacctgattgccctgagcctgggcctgacccccaacttcaagagcaacttcgacctggccgaggatgccaaactgcagctgagcaaggacacctacgacgacgacctggacaacctgctggcccagatcggcgaccagtacgccgacctgtttctggccgccaagaacctgtccgacgccatcctgctgagcgacatcctgagagtgaacaccgagatcaccaaggcccccctgagcgcctctatgatcaagagatacgacgagcaccaccaggacctgaccctgctgaaagctctcgtgcggcagcagctgcctgagaagtacaaagagattttcttcgaccagagcaagaacggctacgccggctacattgacggcggagccagccaggaagagttctacaagttcatcaagcccatcctggaaaagatggacggcaccgaggaactgctcgtgaagctgaacagagaggacctgctgcggaagcagcggaccttcgacaacggcagcatcccccaccagatccacctgggagagctgcacgccattctgcggcggcaggaagatttttacccattcctgaaggacaaccgggaaaagatcgagaagatcctgaccttccgcatcccctactacgtgggccctctggccaggggaaacagcagattcgcctggatgaccagaaagagcgaggaaaccatcaccccctggaacttcgaggaagtggtggacaagggcgcttccgcccagagcttcatcgagcggatgaccaacttcgataagaacctgcccaacgagaaggtgctgcccaagcacagcctgctgtacgagtacttcaccgtgtataacgagctgaccaaagtgaaatacgtgaccgagggaatgagaaagcccgccttcctgagcggcgagcagaaaaaggccatcgtggacctgctgttcaagaccaaccggaaagtgaccgtgaagcagctgaaagaggactacttcaagaaaatcgagtgcttcgactccgtggaaatctccggcgtggaagatcggttcaacgcctccctgggcacataccacgatctgctgaaaattatcaaggacaaggacttcctggacaatgaggaaaacgaggacattctggaagatatcgtgctgaccctgacactgtttgaggacagagagatgatcgaggaacggctgaaaacctatgcccacctgttcgacgacaaagtgatgaagcagctgaagcggcggagatacaccggctggggcaggctgagccggaagctgatcaacggcatccgggacaagcagtccggcaagacaatcctggatttcctgaagtccgacggcttcgccaacagaaacttcatgcagctgatccacgacgacagcctgacctttaaagaggacatccagaaagcccaggtgtccggccagggcgatagcctgcacgagcacattgccaatctggccggcagccccgccattaagaagggcatcctgcagacagtgaaggtggtggacgagctcgtgaaagtgatgggccggcacaagcccgagaacatcgtgatcgaaatggccagagagaaccagaccacccagaagggacagaagaacagccgcgagagaatgaagcggatcgaagagggcatcaaagagctgggcagccagatcctgaaagaacaccccgtggaaaacacccagctgcagaacgagaagctgtacctgtactacctgcagaatgggcgggatatgtacgtggaccaggaactggacatcaaccggctgtccgactacgatgtggaccatatcgtgcctcagagctttctgaaggacgactccatcgacaacaaggtgctgaccagaagcgacaagaaccggggcaagagcgacaacgtgccctccgaagaggtcgtgaagaagatgaagaactactggcggcagctgctgaacgccaagctgattacccagagaaagttcgacaatctgaccaaggccgagagaggcggcctgagcgaactggataaggccggcttcatcaagagacagctggtggaaacccggcagatcacaaagcacgtggcacagatcctggactcccggatgaacactaagtacgacgagaatgacaagctgatccgggaagtgaaagtgatcaccctgaagtccaagctggtgtccgatttccggaaggatttccagttttacaaagtgcgcgagatcaacaactaccaccacgcccacgacgcctacctgaacgccgtcgtgggaaccgccctgatcaaaaagtaccctaagctggaaagcgagttcgtgtacggcgactacaaggtgtacgacgtgcggaagatgatcgccaagagcgagcaggaaatcggcaaggctaccgccaagtacttcttctacagcaacatcatgaactttttcaagaccgagattaccctggccaacggcgagatccggaagcggcctctgatcgagacaaacggcgaaaccggggagatcgtgtgggataagggccgggattttgccaccgtgcggaaagtgctgagcatgccccaagtgaatatcgtgaaaaagaccgaggtgcagacaggcggcttcagcaaagagtctatcctgcccaagaggaacagcgataagctgatcgccagaaagaaggactgggaccctaagaagtacggcggcttcgacagccccaccgtggcctattctgtgctggtggtggccaaagtggaaaagggcaagtccaagaaactgaagagtgtgaaagagctgctggggatcaccatcatggaaagaagcagcttcgagaagaatcccatcgactttctggaagccaagggctacaaagaagtgaaaaaggacctgatcatcaagctgcctaagtactccctgttcgagctggaaaacggccggaagagaatgctggcctctgccggcgaactgcagaagggaaacgaactggccctgccctccaaatatgtgaacttcctgtacctggccagccactatgagaagctgaagggctcccccgaggataatgagcagaaacagctgtttgtggaacagcacaagcactacctggacgagatcatcgagcagatcagcgagttctccaagagagtgatcctggccgacgctaatctggacaaagtgctgtccgcctacaacaagcaccgggataagcccatcagagagcaggccgagaatatcatccacctgtttaccctgaccaatctgggagcccctgccgccttcaagtactttgacaccaccatcgaccggaagaggtacaccagcaccaaagaggtgctggacgccaccctgatccaccagagcatcaccggcctgtacgagacacggatcgacctgtctcagctgggaggcgacaattgtctgggtggcggaggaagcggaggcggcggatctggcggcggaggatccggcggtggtggttctggcggtggcggtagtggcggaggtggtagcggtggtggcggatccaccggcggtgaccattatctggatattcggctgaggcctgatccagagttcccacctgcgcagctgatgtctgtcctttttggcaaacttcatcaggccctggttgcccagggcggagatcggataggggtaagctttccagacctcgacgaaagccggagccgcctgggagaacgcctgcggatccacgcttctgccgacgatctgagagccttgctggcaaggccatggcttgaggggctccgggatcacctgcagtttggcgaacccgccgttgttccccacccaaccccttatcggcaggtgtctagagtgcaggccaaatctaatccagaacggctgcgacggcgactcatgcggcgacatgatcttagcgaggaagaggcccgaaaaagaatccctgataccgtggcccgcgcccttgacttgccttttgtcacactgcggtcccagagtacggggcagcatttcagacttttcattcgacacgggccactgcaagttaccgccgaagaaggaggctttacttgttatggactctccaagggaggtttcgtgccctggtttttcgaaagcgctctcgaggccggcaaaagaaccgccgatggcagcgagtttgagagccctaagaaaaaacggaaggtgtag

SEQ ID NO: 67 - protein, 1837 aa, artificial sequence
  artificial protein C9C4v2 BE1
MKRTADGSEFESPKKKRKVSEVEFSHEYWMRHALTLAKRARDEREVPVGAVLVLNNRVIGEGWNRAIGLHDPTAHAEIMALRQGGLVMQNYRLIDATLYVTFEPCVMCAGAMIHSRIGRVVFGVRNSKRGAAGSLMNVLNYPGMNHRVEITEGILADECAALLCDFYRMPRQVFNAQKKAQSSINSGGSSGGSSGSETPGTSESATPESSGGSSGGSDKKYSIGLAIGTNSVGWAVITDEYKVPSKKFKVLGNTDRHSIKKNLIGALLFDSGETAEATRLKRTARRRYTRRKNRICYLQEIFSNEMAKVDDSFFHRLEESFLVEEDKKHERHPIFGNIVDEVAYHEKYPTIYHLRKKLVDSTDKADLRLIYLALAHMIKFRGHFLIEGDLNPDNSDVDKLFIQLVQTYNQLFEENPINASGVDAKAILSARLSKSRRLENLIAQLPGEKKNGLFGNLIALSLGLTPNFKSNFDLAEDAKLQLSKDTYDDDLDNLLAQIGDQYADLFLAAKNLSDAILLSDILRVNTEITKAPLSASMIKRYDEHHQDLTLLKALVRQQLPEKYKEIFFDQSKNGYAGYIDGGASQEEFYKFIKPILEKMDGTEELLVKLNREDLLRKQRTFDNGSIPHQIHLGELHAILRRQEDFYPFLKDNREKIEKILTFRIPYYVGPLARGNSRFAWMTRKSEETITPWNFEEVVDKGASAQSFIERMTNFDKNLPNEKVLPKHSLLYEYFTVYNELTKVKYVTEGMRKPAFLSGEQKKAIVDLLFKTNRKVTVKQLKEDYFKKIECFDSVEISGVEDRFNASLGTYHDLLKIIKDKDFLDNEENEDILEDIVLTLTLFEDREMIEERLKTYAHLFDDKVMKQLKRRRYTGWGRLSRKLINGIRDKQSGKTILDFLKSDGFANRNFMQLIHDDSLTFKEDIQKAQVSGQGDSLHEHIANLAGSPAIKKGILQTVKVVDELVKVMGRHKPENIVIEMARENQTTQKGQKNSRERMKRIEEGIKELGSQILKEHPVENTQLQNEKLYLYYLQNGRDMYVDQELDINRLSDYDVDHIVPQSFLKDDSIDNKVLTRSDKNRGKSDNVPSEEVVKKMKNYWRQLLNAKLITQRKFDNLTKAERGGLSELDKAGFIKRQLVETRQITKHVAQILDSRMNTKYDENDKLIREVKVITLKSKLVSDFRKDFQFYKVREINNYHHAHDAYLNAVVGTALIKKYPKLESEFVYGDYKVYDVRKMIAKSEQEIGKATAKYFFYSNIMNFFKTEITLANGEIRKRPLIETNGETGEIVWDKGRDFATVRKVLSMPQVNIVKKTEVQTGGFSKESILPKRNSDKLIARKKDWDPKKYGGFDSPTVAYSVLVVAKVEKGKSKKLKSVKELLGITIMERSSFEKNPIDFLEAKGYKEVKKDLIIKLPKYSLFELENGRKRMLASAGELQKGNELALPSKYVNFLYLASHYEKLKGSPEDNEQKQLFVEQHKHYLDEIIEQISEFSKRVILADANLDKVLSAYNKHRDKPIREQAENIIHLFTLTNLGAPAAFKYFDTTIDRKRYTSTKEVLDATLIHQSITGLYETRIDLSQLGGDNCLGGGGSGGGGSGGGGSGGGGSGGGGSGGGGSGGGGSTGGDHYLDIRLRPDPEFPPAQLMSVLFGKLHQALVAQGGDRIGVSFPDLDESRSRLGERLRLHASADDLRALLARPWLEGLRDHLQFGEPAVVPHPTPYRQVSRVQAKSNPERLRRRLMRRHDLSEEEARKRIPDTVARALDLPFVTLRSQSTGQHFRLFIRHGPLQVTAEEGGFTCYGLSKGGFVPWFFESALEAGKRTADGSEFESPKKKRKV

SEQ ID NO: 68 - DNA, 4881 bp, artificial sequence; identical to SEQ ID NO: 64
  DNA sequence encoding artificial protein C9C4v2 BE1

SEQ ID NO: 69 - DNA, 4236 bp, artificial sequence
  DNA sequence encoding C9
atggattacaaagacgatgacgataagatggccccaaagaagaagcggaaggtcggtatccacggagtcccagcagccgacaagaagtacagcatcggcctggacatcggcaccaactctgtgggctgggccgtgatcaccgacgagtacaaggtgcccagcaagaaattcaaggtgctgggcaacaccgaccggcacagcatcaagaagaacctgatcggagccctgctgttcgacagcggcgaaacagccgaggccacccggctgaagagaaccgccagaagaagatacaccagacggaagaaccggatctgctatctgcaagagatcttcagcaacgagatggccaaggtggacgacagcttcttccacagactggaagagtccttcctggtggaagaggataagaagcacgagcggcaccccatcttcggcaacatcgtggacgaggtggcctaccacgagaagtaccccaccatctaccacctgagaaagaaactggtggacagcaccgacaaggccgacctgcggctgatctatctggccctggcccacatgatcaagttccggggccacttcctgatcgagggcgacctgaaccccgacaacagcgacgtggacaagctgttcatccagctggtgcagacctacaaccagctgttcgaggaaaaccccatcaacgccagcggcgtggacgccaaggccatcctgtctgccagactgagcaagagcagacggctggaaaatctgatcgcccagctgcccggcgagaagaagaatggcctgttcggaaacctgattgccctgagcctgggcctgacccccaacttcaagagcaacttcgacctggccgaggatgccaaactgcagctgagcaaggacacctacgacgacgacctggacaacctgctggcccagatcggcgaccagtacgccgacctgtttctggccgccaagaacctgtccgacgccatcctgctgagcgacatcctgagagtgaacaccgagatcaccaaggcccccctgagcgcctctatgatcaagagatacgacgagcaccaccaggacctgaccctgctgaaagctctcgtgcggcagcagctgcctgagaagtacaaagagattttcttcgaccagagcaagaacggctacgccggctacattgacggcggagccagccaggaagagttctacaagttcatcaagcccatcctggaaaagatggacggcaccgaggaactgctcgtgaagctgaacagagaggacctgctgcggaagcagcggaccttcgacaacggcagcatcccccaccagatccacctgggagagctgcacgccattctgcggcggcaggaagatttttacccattcctgaaggacaaccgggaaaagatcgagaagatcctgaccttccgcatcccctactacgtgggccctctggccaggggaaacagcagattcgcctggatgaccagaaagagcgaggaaaccatcaccccctggaacttcgaggaagtggtggacaagggcgcttccgcccagagcttcatcgagcggatgaccaacttcgataagaacctgcccaacgagaaggtgctgcccaagcacagcctgctgtacgagtacttcaccgtgtataacgagctgaccaaagtgaaatacgtgaccgagggaatgagaaagcccgccttcctgagcggcgagcagaaaaaggccatcgtggacctgctgttcaagaccaaccggaaagtgaccgtgaagcagctgaaagaggactacttcaagaaaatcgagtgcttcgactccgtggaaatctccggcgtggaagatcggttcaacgcctccctgggcacataccacgatctgctgaaaattatcaaggacaaggacttcctggacaatgaggaaaacgaggacattctggaagatatcgtgctgaccctgacactgtttgaggacagagagatgatcgaggaacggctgaaaacctatgcccacctgttcgacgacaaagtgatgaagcagctgaagcggcggagatacaccggctggggcaggctgagccggaagctgatcaacggcatccgggacaagcagtccggcaagacaatcctggatttcctgaagtccgacggcttcgccaacagaaacttcatgcagctgatccacgacgacagcctgacctttaaagaggacatccagaaagcccaggtgtccggccagggcgatagcctgcacgagcacattgccaatctggccggcagccccgccattaagaagggcatcctgcagacagtgaaggtggtggacgagctcgtgaaagtgatgggccggcacaagcccgagaacatcgtgatcgaaatggccagagagaaccagaccacccagaagggacagaagaacagccgcgagagaatgaagcggatcgaagagggcatcaaagagctgggcagccagatcctgaaagaacaccccgtggaaaacacccagctgcagaacgagaagctgtacctgtactacctgcagaatgggcgggatatgtacgtggaccaggaactggacatcaaccggctgtccgactacgatgtggaccatatcgtgcctcagagctttctgaaggacgactccatcgacaacaaggtgctgaccagaagcgacaagaaccggggcaagagcgacaacgtgccctccgaagaggtcgtgaagaagatgaagaactactggcggcagctgctgaacgccaagctgattacccagagaaagttcgacaatctgaccaaggccgagagaggcggcctgagcgaactggataaggccggcttcatcaagagacagctggtggaaacccggcagatcacaaagcacgtggcacagatcctggactcccggatgaacactaagtacgacgagaatgacaagctgatccgggaagtgaaagtgatcaccctgaagtccaagctggtgtccgatttccggaaggatttccagttttacaaagtgcgcgagatcaacaactaccaccacgcccacgacgcctacctgaacgccgtcgtgggaaccgccctgatcaaaaagtaccctaagctggaaagcgagttcgtgtacggcgactacaaggtgtacgacgtgcggaagatgatcgccaagagcgagcaggaaatcggcaaggctaccgccaagtacttcttctacagcaacatcatgaactttttcaagaccgagattaccctggccaacggcgagatccggaagcggcctctgatcgagacaaacggcgaaaccggggagatcgtgtgggataagggccgggattttgccaccgtgcggaaagtgctgagcatgccccaagtgaatatcgtgaaaaagaccgaggtgcagacaggcggcttcagcaaagagtctatcctgcccaagaggaacagcgataagctgatcgccagaaagaaggactgggaccctaagaagtacggcggcttcgacagccccaccgtggcctattctgtgctggtggtggccaaagtggaaaagggcaagtccaagaaactgaagagtgtgaaagagctgctggggatcaccatcatggaaagaagcagcttcgagaagaatcccatcgactttctggaagccaagggctacaaagaagtgaaaaaggacctgatcatcaagctgcctaagtactccctgttcgagctggaaaacggccggaagagaatgctggcctctgccggcgaactgcagaagggaaacgaactggccctgccctccaaatatgtgaacttcctgtacctggccagccactatgagaagctgaagggctcccccgaggataatgagcagaaacagctgtttgtggaacagcacaagcactacctggacgagatcatcgagcagatcagcgagttctccaagagagtgatcctggccgacgctaatctggacaaagtgctgtccgcctacaacaagcaccgggataagcccatcagagagcaggccgagaatatcatccacctgtttaccctgaccaatctgggagcccctgccgccttcaagtactttgacaccaccatcgaccggaagaggtacaccagcaccaaagaggtgctggacgccaccctgatccaccagagcatcaccggcctgtacgagacacggatcgacctgtctcagctgggaggcgacaagcgtcctgctgctactaagaaagctggtcaagctaagaaaaagaaagctagctga

SEQ ID NO: 70 - DNA, 5025 bp, artificial sequence
  DNA sequence encoding C9-GFP
atggattacaaagacgatgacgataagatggccccaaagaagaagcggaaggtcggtatccacggagtcccagcagccgacaagaagtacagcatcggcctggacatcggcaccaactctgtgggctgggccgtgatcaccgacgagtacaaggtgcccagcaagaaattcaaggtgctgggcaacaccgaccggcacagcatcaagaagaacctgatcggagccctgctgttcgacagcggcgaaacagccgaggccacccggctgaagagaaccgccagaagaagatacaccagacggaagaaccggatctgctatctgcaagagatcttcagcaacgagatggccaaggtggacgacagcttcttccacagactggaagagtccttcctggtggaagaggataagaagcacgagcggcaccccatcttcggcaacatcgtggacgaggtggcctaccacgagaagtaccccaccatctaccacctgagaaagaaactggtggacagcaccgacaaggccgacctgcggctgatctatctggccctggcccacatgatcaagttccggggccacttcctgatcgagggcgacctgaaccccgacaacagcgacgtggacaagctgttcatccagctggtgcagacctacaaccagctgttcgaggaaaaccccatcaacgccagcggcgtggacgccaaggccatcctgtctgccagactgagcaagagcagacggctggaaaatctgatcgcccagctgcccggcgagaagaagaatggcctgttcggcaacctgattgccctgagcctgggcctgacccccaacttcaagagcaacttcgacctggccgaggatgccaaactgcagctgagcaaggacacctacgacgacgacctggacaacctgctggcccagatcggcgaccagtacgccgacctgtttctggccgccaagaacctgtccgacgccatcctgctgagcgacatcctgagagtgaacaccgagatcaccaaggcccccctgagcgcctctatgatcaagagatacgacgagcaccaccaggacctgaccctgctgaaagctctcgtgcggcagcagctgcctgagaagtacaaagagattttcttcgaccagagcaagaacggctacgccggctacattgacggcggagccagccaggaagagttctacaagttcatcaagcccatcctggaaaagatggacggcaccgaggaactgctcgtgaagctgaacagagaggacctgctgcggaagcagcggaccttcgacaacggcagcatcccccaccagatccacctgggagagctgcacgccattctgcggcggcaggaagatttttacccattcctgaaggacaaccgggaaaagatcgagaagatcctgaccttccgcatcccctactacgtgggccctctggccaggggaaacagcagattcgcctggatgaccagaaagagcgaggaaaccatcaccccctggaacttcgaggaagtggtggacaagggcgcttccgcccagagcttcatcgagcggatgaccaacttcgataagaacctgcccaacgagaaggtgctgcccaagcacagcctgctgtacgagtacttcaccgtgtataacgagctgaccaaagtgaaatacgtgaccgagggaatgagaaagcccgccttcctgagcggcgagcagaaaaaggccatcgtggacctgctgttcaagaccaaccggaaagtgaccgtgaagcagctgaaagaggactacttcaagaaaatcgagtgcttcgactccgtggaaatctccggcgtggaagatcggttcaacgcctccctgggcacataccacgatctgctgaaaattatcaaggacaaggacttcctggacaatgaggaaaacgaggacattctggaagatatcgtgctgaccctgacactgtttgaggacagagagatgatcgaggaacggctgaaaacctatgcccacctgttcgacgacaaagtgatgaagcagctgaagcggcggagatacaccggctggggcaggctgagccggaagctgatcaacggcatccgggacaagcagtccggcaagacaatcctggatttcctgaagtccgacggcttcgccaacagaaacttcatgcagctgatccacgacgacagcctgacctttaaagaggacatccagaaagcccaggtgtccggccagggcgatagcctgcacgagcacattgccaatctggccggcagccccgccattaagaagggcatcctgcagacagtgaaggtggtggacgagctcgtgaaagtgatgggccggcacaagcccgagaacatcgtgatcgaaatggccagagagaaccagaccacccagaagggacagaagaacagccgcgagagaatgaagcggatcgaagagggcatcaaagagctgggcagccagatcctgaaagaacaccccgtggaaaacacccagctgcagaacgagaagctgtacctgtactacctgcagaatgggcgggatatgtacgtggaccaggaactggacatcaaccggctgtccgactacgatgtggaccatatcgtgcctcagagctttctgaaggacgactccatcgacaacaaggtgctgaccagaagcgacaagaaccggggcaagagcgacaacgtgccctccgaagaggtcgtgaagaagatgaagaactactggcggcagctgctgaacgccaagctgattacccagagaaagttcgacaatctgaccaaggccgagagaggcggcctgagcgaactggataaggccggcttcatcaagagacagctggtggaaacccggcagatcacaaagcacgtggcacagatcctggactcccggatgaacactaagtacgacgagaatgacaagctgatccgggaagtgaaagtgatcaccctgaagtccaagctggtgtccgatttccggaaggatttccagttttacaaagtgcgcgagatcaacaactaccaccacgcccacgacgcctacctgaacgccgtcgtgggaaccgccctgatcaaaaagtaccctaagctggaaagcgagttcgtgtacggcgactacaaggtgtacgacgtgcggaagatgatcgccaagagcgagcaggaaatcggcaaggctaccgccaagtacttcttctacagcaacatcatgaactttttcaagaccgagattaccctggccaacggcgagatccggaagcggcctctgatcgagacaaacggcgaaaccggggagatcgtgtgggataagggccgggattttgccaccgtgcggaaagtgctgagcatgccccaagtgaatatcgtgaaaaagaccgaggtgcagacaggcggcttcagcaaagagtctatcctgcccaagaggaacagcgataagctgatcgccagaaagaaggactgggaccctaagaagtacggcggcttcgacagccccaccgtggcctattctgtgctggtggtggccaaagtggaaaagggcaagtccaagaaactgaagagtgtgaaagagctgctggggatcaccatcatggaaagaagcagcttcgagaagaatcccatcgactttctggaagccaagggctacaaagaagtgaaaaaggacctgatcatcaagctgcctaagtactccctgttcgagctggaaaacggccggaagagaatgctggcctctgccggcgaactgcagaagggaaacgaactggccctgccctccaaatatgtgaacttcctgtacctggccagccactatgagaagctgaagggctcccccgaggataatgagcagaaacagctgtttgtggaacagcacaagcactacctggacgagatcatcgagcagatcagcgagttctccaagagagtgatcctggccgacgctaatctggacaaagtgctgtccgcctacaacaagcaccgggataagcccatcagagagcaggccgagaatatcatccacctgtttaccctgaccaatctgggagcccctgccgccttcaagtactttgacaccaccatcgaccggaagaggtacaccagcaccaaagaggtgctggacgccaccctgatccaccagagcatcaccggcctgtacgagacacggatcgacctgtctcagctgggaggcgacaagcgtcctgctgctactaagaaagctggtcaagctaagaaaaagaaagctagcggcagcggcatgcagttcgaaggcagaggctccctgctgacctgcggcgacgtggaggagaaccccgggcccatggtgagcaagggcgaggagctgttcaccggggtggtgcccatcctggtcgagctggacggcgacgtaaacggccacaagttcagcgtgtccggcgagggcgagggcgatgccacctacggcaagctgaccctgaagttcatctgcaccaccggcaagctgcccgtgccctggcccaccctcgtgaccaccctgacctacggcgtgcagtgcttcagccgctaccccgatcacatgaagcagcacgacttcttcaagtccgccatgcccgaaggctacgtccaggagcgcacgatcttcttcaaggacgacggcaactacaagacccgcgccgaggtgaagttcgagggcgacaccctggtgaaccgcatcgagctgaagggcatcgacttcaaggaggacggcaacatcctggggcacaagctggagtacaactacaacagccacaacgtctatatcatggccgacaagcagaagaacggcatcaaggtgaacttcaagatccgccacaacatcgaggacggcagcgtgcagctcgccgaccactaccagcagaacacccccatcggcgacggccccgtgctgctgcccgacaaccactacctgagcacccagtccgccctgagcaaagaccccaacgagaagcgcgatcacatggtcctgctggagttcgtgaccgccgccgggatcactctcggcatggacgagctgtacaagtga

SEQ ID NO: 71 - DNA, 4833 bp, artificial sequence
  DNA sequence encoding C4-C9
atgggtgatcattatctggatattcggctgaggcctgatccagagttcccacctgcgcagctgatgtctgtcctttttggcaaacttcatcaggccctggttgcccagggcggagatcggataggggtaagctttccagacctcgacgaaagccggagccgcctgggagaacgcctgcggatccacgcttctgccgacgatctgagagccttgctggcaaggccatggcttgaggggctccgggatcacctgcagtttggcgaacccgccgttgttccccacccaaccccttatcggcaggtgtctagagtgcaggccaaatctaatccagaacggctgcgacggcgactcatgcggcgacatgatcttagcgaggaagaggcccgaaaaagaatccctgataccgtggcccgcgcccttgacttgccttttgtcacactgcggtcccagagtacggggcagcatttcagacttttcattcgacacgggccactgcaagttaccgccgaagaaggaggctttacttgttatggactctccaagggaggtttcgtgccctggtttttcgaaggcagaggctccctgctgacctgcggcgacgtggaggagaaccccgggcctaggatggccccaaagaagaagcggaaggtcggtatccacggagtcccagcagccgacaagaagtacagcatcggcctggacatcggcaccaactctgtgggctgggccgtgatcaccgacgagtacaaggtgcccagcaagaaattcaaggtgctgggcaacaccgaccggcacagcatcaagaagaacctgatcggagccctgctgttcgacagcggcgaaacagccgaggccacccggctgaagagaaccgccagaagaagatacaccagacggaagaaccggatctgctatctgcaagagatcttcagcaacgagatggccaaggtggacgacagcttcttccacagactggaagagtccttcctggtggaagaggataagaagcacgagcggcaccccatcttcggcaacatcgtggacgaggtggcctaccacgagaagtaccccaccatctaccacctgagaaagaaactggtggacagcaccgacaaggccgacctgcggctgatctatctggccctggcccacatgatcaagttccggggccacttcctgatcgagggcgacctgaaccccgacaacagcgacgtggacaagctgttcatccagctggtgcagacctacaaccagctgttcgaggaaaaccccatcaacgccagcggcgtggacgccaaggccatcctgtctgccagactgagcaagagcagacggctggaaaatctgatcgcccagctgcccggcgagaagaagaatggcctgttcggaaacctgattgccctgagcctgggcctgacccccaacttcaagagcaacttcgacctggccgaggatgccaaactgcagctgagcaaggacacctacgacgacgacctggacaacctgctggcccagatcggcgaccagtacgccgacctgtttctggccgccaagaacctgtccgacgccatcctgctgagcgacatcctgagagtgaacaccgagatcaccaaggcccccctgagcgcctctatgatcaagagatacgacgagcaccaccaggacctgaccctgctgaaagctctcgtgcggcagcagctgcctgagaagtacaaagagattttcttcgaccagagcaagaacggctacgccggctacattgacggcggagccagccaggaagagttctacaagttcatcaagcccatcctggaaaagatggacggcaccgaggaactgctcgtgaagctgaacagagaggacctgctgcggaagcagcggaccttcgacaacggcagcatcccccaccagatccacctgggagagctgcacgccattctgcggcggcaggaagatttttacccattcctgaaggacaaccgggaaaagatcgagaagatcctgaccttccgcatcccctactacgtgggccctctggccaggggaaacagcagattcgcctggatgaccagaaagagcgaggaaaccatcaccccctggaacttcgaggaagtggtggacaagggcgcttccgcccagagcttcatcgagcggatgaccaacttcgataagaacctgcccaacgagaaggtgctgcccaagcacagcctgctgtacgagtacttcaccgtgtataacgagctgaccaaagtgaaatacgtgaccgagggaatgagaaagcccgccttcctgagcggcgagcagaaaaaggccatcgtggacctgctgttcaagaccaaccggaaagtgaccgtgaagcagctgaaagaggactacttcaagaaaatcgagtgcttcgactccgtggaaatctccggcgtggaagatcggttcaacgcctccctgggcacataccacgatctgctgaaaattatcaaggacaaggacttcctggacaatgaggaaaacgaggacattctggaagatatcgtgctgaccctgacactgtttgaggacagagagatgatcgaggaacggctgaaaacctatgcccacctgttcgacgacaaagtgatgaagcagctgaagcggcggagatacaccggctggggcaggctgagccggaagctgatcaacggcatccgggacaagcagtccggcaagacaatcctggatttcctgaagtccgacggcttcgccaacagaaacttcatgcagctgatccacgacgacagcctgacctttaaagaggacatccagaaagcccaggtgtccggccagggcgatagcctgcacgagcacattgccaatctggccggcagccccgccattaagaagggcatcctgcagacagtgaaggtggtggacgagctcgtgaaagtgatgggccggcacaagcccgagaacatcgtgatcgaaatggccagagagaaccagaccacccagaagggacagaagaacagccgcgagagaatgaagcggatcgaagagggcatcaaagagctgggcagccagatcctgaaagaacaccccgtggaaaacacccagctgcagaacgagaagctgtacctgtactacctgcagaatgggcgggatatgtacgtggaccaggaactggacatcaaccggctgtccgactacgatgtggaccatatcgtgcctcagagctttctgaaggacgactccatcgacaacaaggtgctgaccagaagcgacaagaaccggggcaagagcgacaacgtgccctccgaagaggtcgtgaagaagatgaagaactactggcggcagctgctgaacgccaagctgattacccagagaaagttcgacaatctgaccaaggccgagagaggcggcctgagcgaactggataaggccggcttcatcaagagacagctggtggaaacccggcagatcacaaagcacgtggcacagatcctggactcccggatgaacactaagtacgacgagaatgacaagctgatccgggaagtgaaagtgatcaccctgaagtccaagctggtgtccgatttccggaaggatttccagttttacaaagtgcgcgagatcaacaactaccaccacgcccacgacgcctacctgaacgccgtcgtgggaaccgccctgatcaaaaagtaccctaagctggaaagcgagttcgtgtacggcgactacaaggtgtacgacgtgcggaagatgatcgccaagagcgagcaggaaatcggcaaggctaccgccaagtacttcttctacagcaacatcatgaactttttcaagaccgagattaccctggccaacggcgagatccggaagcggcctctgatcgagacaaacggcgaaaccggggagatcgtgtgggataagggccgggattttgccaccgtgcggaaagtgctgagcatgccccaagtgaatatcgtgaaaaagaccgaggtgcagacaggcggcttcagcaaagagtctatcctgcccaagaggaacagcgataagctgatcgccagaaagaaggactgggaccctaagaagtacggcggcttcgacagccccaccgtggcctattctgtgctggtggtggccaaagtggaaaagggcaagtccaagaaactgaagagtgtgaaagagctgctggggatcaccatcatggaaagaagcagcttcgagaagaatcccatcgactttctggaagccaagggctacaaagaagtgaaaaaggacctgatcatcaagctgcctaagtactccctgttcgagctggaaaacggccggaagagaatgctggcctctgccggcgaactgcagaagggaaacgaactggccctgccctccaaatatgtgaacttcctgtacctggccagccactatgagaagctgaagggctcccccgaggataatgagcagaaacagctgtttgtggaacagcacaagcactacctggacgagatcatcgagcagatcagcgagttctccaagagagtgatcctggccgacgctaatctggacaaagtgctgtccgcctacaacaagcaccgggataagcccatcagagagcaggccgagaatatcatccacctgtttaccctgaccaatctgggagcccctgccgccttcaagtactttgacaccaccatcgaccggaagaggtacaccagcaccaaagaggtgctggacgccaccctgatccaccagagcatcaccggcctgtacgagacacggatcgacctgtctcagctgggaggcgacaagcgtcctgctgctactaagaaagctggtcaagctaagaaaaagaaagctagctga

SEQ ID NO: 72 - RNA, 100 nt, artificial sequence
  IDPV C9-gfp-148 sgRNA, TraFo C9-gfp-148 sgRNA
gggcacgggcagcuugccggguuuuagagcuagaaauagcaaguuaaaauaaggcuaguccguuaucaacuugaaaaaguggcaccgagucggugcuuuu

SEQ ID NO: 73 - DNA, 100 bp, artificial sequence
  DNA sequence encoding IDPV C9-gfp-148 sgRNA, DNA sequence encoding TraFo C9-gfp-148 sgRNA
gggcacgggcagcttgccgggttttagagctagaaatagcaagttaaaataaggctagtccgttatcaacttgaaaaagtggcaccgagtcggtgctttt

SEQ ID NO: 74 - RNA, 1693 nt, artificial sequence
  pre-C4/C9-gfp+174-112 sgRNA
gucagaucgccugcagacgccauccacgcuguuuugaccuccauagaagacaccgggaccgauccagccuccgcggccgggaacggugcauuggaacgcggauuccccgugccaagagugacucaccguccuugacacgaagcuugcuagcgcuaccggacucagauccaccggucgccaccauggauagcacugagaacgucaucaagcccuucaugcgcuucaaggugcacauggagggcuccgugaacggccacgaguucgagaucgagggcgagggcgagggcaagcccuacgagggcacccagaccgccaagcugcaggugaccaagggcggcccccugcccuucgccugggacauccuguccccccaguuccaguacggcuccaagguguacgugaagcaccccgccgacauccccgacuacaagaagcuguccuuccccgagggcuucaagugggagcgcgugaugaacuucgaggacggcggcguggugaccgugacccaggacuccucccugcaggacggcaccuucaucuaccacgugaaguucaucggcgugaacuuccccuccgacggccccguaaugcagaagaagacucugggcugggagcccuccaccgagcgccuguacccccgcgacggcgugcugaagggcgagauccacaaggcgcugaagcugaagggcggcggccacuaccugguggaguucaagucaaucuacauggccaagaagcccgugaagcugcccggcuacuacuacguggacuccaagcuggacaucaccucccacaacgaggacuacaccgugguggagcaguacgagcgcgccgaggcccgccaccaccuguuccaguaggguaccgagcucggauccacuaguccagugugguggaauucguucacugccguauaggcagccggcaagcugcccgugcccguuuuagagcuagaaauagcaaguuaaaauaaggcuaguccguuaucaacuugaaaaaguggcaccgagucggugcguucacugccguauaggcacagggucagcuugccguaggguuuuagagcuagaaauagcaaguuaaaauaaggcuaguccguuaucaacuugaaaaaguggcaccgagucggugcguucacugccguauaggcagcggccgcgucgacaaucaaccucuggauuacaaaauuugugaaagauugacugguauucuuaacuauguugcuccuuuuacgcuauguggauacgcugcuuuaaugccuuuguaucaugcuauugcuucccguauggcuuucauuuucuccuccuuguauaaauccugguugcugucucuuuaugaggaguuguggcccguugucaggcaacguggcguggugugcacuguguuugcugacgcaacccccacugguuggggcauugccaccaccugucagcuccuuuccgggacuuucgcuuucccccucccuauugccacggcggaacucaucgccgccugccuugcccgcugcuggacaggggcucggcuguugggcacugacaauuccgugguguugucucgaaacccgcugaucagccucgacugugccuucuaguugccagccaucuguuguuugccccucccccgugccuuccuugacccuggaaggugccacucccacuguccuuuccuaauaaaaugaggaaauugcaucgca

SEQ ID NO: 75 - DNA, 1693 bp, artificial sequence
  DNA sequence encoding pre-C4/C9-gfp+174-112 sgRNA
gtcagatcgcctgcagacgccatccacgctgttttgacctccatagaagacaccgggaccgatccagcctccgcggccgggaacggtgcattggaacgcggattccccgtgccaagagtgactcaccgtccttgacacgaagcttgctagcgctaccggactcagatccaccggtcgccaccatggatagcactgagaacgtcatcaagcccttcatgcgcttcaaggtgcacatggagggctccgtgaacggccacgagttcgagatcgagggcgagggcgagggcaagccctacgagggcacccagaccgccaagctgcaggtgaccaagggcggccccctgcccttcgcctgggacatcctgtccccccagttccagtacggctccaaggtgtacgtgaagcaccccgccgacatccccgactacaagaagctgtccttccccgagggcttcaagtgggagcgcgtgatgaacttcgaggacggcggcgtggtgaccgtgacccaggactcctccctgcaggacggcaccttcatctaccacgtgaagttcatcggcgtgaacttcccctccgacggccccgtaatgcagaagaagactctgggctgggagccctccaccgagcgcctgtacccccgcgacggcgtgctgaagggcgagatccacaaggcgctgaagctgaagggcggcggccactacctggtggagttcaagtcaatctacatggccaagaagcccgtgaagctgcccggctactactacgtggactccaagctggacatcacctcccacaacgaggactacaccgtggtggagcagtacgagcgcgccgaggcccgccaccacctgttccagtagggtaccgagctcggatccactagtccagtgtggtggaattcgttcactgccgtataggcagccggcaagctgcccgtgcccgttttagagctagaaatagcaagttaaaataaggctagtccgttatcaacttgaaaaagtggcaccgagtcggtgcgttcactgccgtataggcacagggtcagcttgccgtagggttttagagctagaaatagcaagttaaaataaggctagtccgttatcaacttgaaaaagtggcaccgagtcggtgcgttcactgccgtataggcagcggccgcgtcgacaatcaacctctggattacaaaatttgtgaaagattgactggtattcttaactatgttgctccttttacgctatgtggatacgctgctttaatgcctttgtatcatgctattgcttcccgtatggctttcattttctcctccttgtataaatcctggttgctgtctctttatgaggagttgtggcccgttgtcaggcaacgtggcgtggtgtgcactgtgtttgctgacgcaacccccactggttggggcattgccaccacctgtcagctcctttccgggactttcgctttccccctccctattgccacggcggaactcatcgccgcctgccttgcccgctgctggacaggggctcggctgttgggcactgacaattccgtggtgttgtctcgaaacccgctgatcagcctcgactgtgccttctagttgccagccatctgttgtttgcccctcccccgtgccttccttgaccctggaaggtgccactcccactgtcctttcctaataaaatgaggaaattgcatcgca

SEQ ID NO: 76 - RNA, 1578 nt, artificial sequence
  pre-C4/C9-gfp-148 sgRNA
gucagaucgccugcagacgccauccacgcuguuuugaccuccauagaagacaccgggaccgauccagccuccgcggccgggaacggugcauuggaacgcggauuccccgugccaagagugacucaccguccuugacacgaagcuugcuagcgcuaccggacucagauccaccggucgccaccauggauagcacugagaacgucaucaagcccuucaugcgcuucaaggugcacauggagggcuccgugaacggccacgaguucgagaucgagggcgagggcgagggcaagcccuacgagggcacccagaccgccaagcugcaggugaccaagggcggcccccugcccuucgccugggacauccuguccccccaguuccaguacggcuccaagguguacgugaagcaccccgccgacauccccgacuacaagaagcuguccuuccccgagggcuucaagugggagcgcgugaugaacuucgaggacggcggcguggugaccgugacccaggacuccucccugcaggacggcaccuucaucuaccacgugaaguucaucggcgugaacuuccccuccgacggccccguaaugcagaagaagacucugggcugggagcccuccaccgagcgccuguacccccgcgacggcgugcugaagggcgagauccacaaggcgcugaagcugaagggcggcggccacuaccugguggaguucaagucaaucuacauggccaagaagcccgugaagcugcccggcuacuacuacguggacuccaagcuggacaucaccucccacaacgaggacuacaccgugguggagcaguacgagcgcgccgaggcccgccaccaccuguuccaguaggguaccgagcucggauccacuaguccagugugguggaauucguucacugccguauaggcaggggcacgggcagcuugccggguuuuagagcuagaaauagcaaguuaaaauaaggcuaguccguuaucaacuugaaaaaguggcaccgagucggugcguucacugccguauaggcagcggccgcgucgacaaucaaccucuggauuacaaaauuugugaaagauugacugguauucuuaacuauguugcuccuuuuacgcuauguggauacgcugcuuuaaugccuuuguaucaugcuauugcuucccguauggcuuucauuuucuccuccuuguauaaauccugguugcugucucuuuaugaggaguuguggcccguugucaggcaacguggcguggugugcacuguguuugcugacgcaacccccacugguuggggcauugccaccaccugucagcuccuuuccgggacuuucgcuuucccccucccuauugccacggcggaacucaucgccgccugccuugcccgcugcuggacaggggcucggcuguugggcacugacaauuccgugguguugucucgaaacccgcugaucagccucgacugugccuucuaguugccagccaucuguuguuugccccucccccgugccuuccuugacccuggaaggugccacucccacuguccuuuccuaauaaaaugaggaaauugcaucgca

SEQ ID NO: 77 - DNA, 1578 bp, artificial sequence
  DNA sequence encoding pre-C4/C9-gfp-148 sgRNA
gtcagatcgcctgcagacgccatccacgctgttttgacctccatagaagacaccgggaccgatccagcctccgcggccgggaacggtgcattggaacgcggattccccgtgccaagagtgactcaccgtccttgacacgaagcttgctagcgctaccggactcagatccaccggtcgccaccatggatagcactgagaacgtcatcaagcccttcatgcgcttcaaggtgcacatggagggctccgtgaacggccacgagttcgagatcgagggcgagggcgagggcaagccctacgagggcacccagaccgccaagctgcaggtgaccaagggcggccccctgcccttcgcctgggacatcctgtccccccagttccagtacggctccaaggtgtacgtgaagcaccccgccgacatccccgactacaagaagctgtccttccccgagggcttcaagtgggagcgcgtgatgaacttcgaggacggcggcgtggtgaccgtgacccaggactcctccctgcaggacggcaccttcatctaccacgtgaagttcatcggcgtgaacttcccctccgacggccccgtaatgcagaagaagactctgggctgggagccctccaccgagcgcctgtacccccgcgacggcgtgctgaagggcgagatccacaaggcgctgaagctgaagggcggcggccactacctggtggagttcaagtcaatctacatggccaagaagcccgtgaagctgcccggctactactacgtggactccaagctggacatcacctcccacaacgaggactacaccgtggtggagcagtacgagcgcgccgaggcccgccaccacctgttccagtagggtaccgagctcggatccactagtccagtgtggtggaattcgttcactgccgtataggcaggggcacgggcagcttgccgggttttagagctagaaatagcaagttaaaataaggctagtccgttatcaacttgaaaaagtggcaccgagtcggtgcgttcactgccgtataggcagcggccgcgtcgacaatcaacctctggattacaaaatttgtgaaagattgactggtattcttaactatgttgctccttttacgctatgtggatacgctgctttaatgcctttgtatcatgctattgcttcccgtatggctttcattttctcctccttgtataaatcctggttgctgtctctttatgaggagttgtggcccgttgtcaggcaacgtggcgtggtgtgcactgtgtttgctgacgcaacccccactggttggggcattgccaccacctgtcagctcctttccgggactttcgctttccccctccctattgccacggcggaactcatcgccgcctgccttgcccgctgctggacaggggctcggctgttgggcactgacaattccgtggtgttgtctcgaaacccgctgatcagcctcgactgtgccttctagttgccagccatctgttgtttgcccctcccccgtgccttccttgaccctggaaggtgccactcccactgtcctttcctaataaaatgaggaaattgcatcgca

SEQ ID NO: 78 - RNA, 1578 nt, artificial sequence
  pre-C4/C9-gfp-197 sgRNA
gucagaucgccugcagacgccauccacgcuguuuugaccuccauagaagacaccgggaccgauccagccuccgcggccgggaacggugcauuggaacgcggauuccccgugccaagagugacucaccguccuugacacgaagcuugcuagcgcuaccggacucagauccaccggucgccaccauggauagcacugagaacgucaucaagcccuucaugcgcuucaaggugcacauggagggcuccgugaacggccacgaguucgagaucgagggcgagggcgagggcaagcccuacgagggcacccagaccgccaagcugcaggugaccaagggcggcccccugcccuucgccugggacauccuguccccccaguuccaguacggcuccaagguguacgugaagcaccccgccgacauccccgacuacaagaagcuguccuuccccgagggcuucaagugggagcgcgugaugaacuucgaggacggcggcguggugaccgugacccaggacuccucccugcaggacggcaccuucaucuaccacgugaaguucaucggcgugaacuuccccuccgacggccccguaaugcagaagaagacucugggcugggagcccuccaccgagcgccuguacccccgcgacggcgugcugaagggcgagauccacaaggcgcugaagcugaagggcggcggccacuaccugguggaguucaagucaaucuacauggccaagaagcccgugaagcugcccggcuacuacuacguggacuccaagcuggacaucaccucccacaacgaggacuacaccgugguggagcaguacgagcgcgccgaggcccgccaccaccuguuccaguaggguaccgagcucggauccacuaguccagugugguggaauucguucacugccguauaggcaggcugaagcacugcacgccguguuuuagagcuagaaauagcaaguuaaaauaaggcuaguccguuaucaacuugaaaaaguggcaccgagucggugcguucacugccguauaggcagcggccgcgucgacaaucaaccucuggauuacaaaauuugugaaagauugacugguauucuuaacuauguugcuccuuuuacgcuauguggauacgcugcuuuaaugccuuuguaucaugcuauugcuucccguauggcuuucauuuucuccuccuuguauaaauccugguugcugucucuuuaugaggaguuguggcccguugucaggcaacguggcguggugugcacuguguuugcugacgcaacccccacugguuggggcauugccaccaccugucagcuccuuuccgggacuuucgcuuucccccucccuauugccacggcggaacucaucgccgccugccuugcccgcugcuggacaggggcucggcuguugggcacugacaauuccgugguguugucucgaaacccgcugaucagccucgacugugccuucuaguugccagccaucuguuguuugccccucccccgugccuuccuugacccuggaaggugccacucccacuguccuuuccuaauaaaaugaggaaauugcaucgca

SEQ ID NO: 79 - DNA, 1578 bp, artificial sequence
  DNA sequence encoding pre-C4/C9-gfp-197 sgRNA
gtcagatcgcctgcagacgccatccacgctgttttgacctccatagaagacaccgggaccgatccagcctccgcggccgggaacggtgcattggaacgcggattccccgtgccaagagtgactcaccgtccttgacacgaagcttgctagcgctaccggactcagatccaccggtcgccaccatggatagcactgagaacgtcatcaagcccttcatgcgcttcaaggtgcacatggagggctccgtgaacggccacgagttcgagatcgagggcgagggcgagggcaagccctacgagggcacccagaccgccaagctgcaggtgaccaagggcggccccctgcccttcgcctgggacatcctgtccccccagttccagtacggctccaaggtgtacgtgaagcaccccgccgacatccccgactacaagaagctgtccttccccgagggcttcaagtgggagcgcgtgatgaacttcgaggacggcggcgtggtgaccgtgacccaggactcctccctgcaggacggcaccttcatctaccacgtgaagttcatcggcgtgaacttcccctccgacggccccgtaatgcagaagaagactctgggctgggagccctccaccgagcgcctgtacccccgcgacggcgtgctgaagggcgagatccacaaggcgctgaagctgaagggcggcggccactacctggtggagttcaagtcaatctacatggccaagaagcccgtgaagctgcccggctactactacgtggactccaagctggacatcacctcccacaacgaggactacaccgtggtggagcagtacgagcgcgccgaggcccgccaccacctgttccagtagggtaccgagctcggatccactagtccagtgtggtggaattcgttcactgccgtataggcaggctgaagcactgcacgccgtgttttagagctagaaatagcaagttaaaataaggctagtccgttatcaacttgaaaaagtggcaccgagtcggtgcgttcactgccgtataggcagcggccgcgtcgacaatcaacctctggattacaaaatttgtgaaagattgactggtattcttaactatgttgctccttttacgctatgtggatacgctgctttaatgcctttgtatcatgctattgcttcccgtatggctttcattttctcctccttgtataaatcctggttgctgtctctttatgaggagttgtggcccgttgtcaggcaacgtggcgtggtgtgcactgtgtttgctgacgcaacccccactggttggggcattgccaccacctgtcagctcctttccgggactttcgctttccccctccctattgccacggcggaactcatcgccgcctgccttgcccgctgctggacaggggctcggctgttgggcactgacaattccgtggtgttgtctcgaaacccgctgatcagcctcgactgtgccttctagttgccagccatctgttgtttgcccctcccccgtgccttccttgaccctggaaggtgccactcccactgtcctttcctaataaaatgaggaaattgcatcgca

SEQ ID NO: 80 - RNA, 1578 nt, artificial sequence
  pre-C4/C9-stuffer sgRNA
gucagaucgccugcagacgccauccacgcuguuuugaccuccauagaagacaccgggaccgauccagccuccgcggccgggaacggugcauuggaacgcggauuccccgugccaagagugacucaccguccuugacacgaagcuugcuagcgcuaccggacucagauccaccggucgccaccauggauagcacugagaacgucaucaagcccuucaugcgcuucaaggugcacauggagggcuccgugaacggccacgaguucgagaucgagggcgagggcgagggcaagcccuacgagggcacccagaccgccaagcugcaggugaccaagggcggcccccugcccuucgccugggacauccuguccccccaguuccaguacggcuccaagguguacgugaagcaccccgccgacauccccgacuacaagaagcuguccuuccccgagggcuucaagugggagcgcgugaugaacuucgaggacggcggcguggugaccgugacccaggacuccucccugcaggacggcaccuucaucuaccacgugaaguucaucggcgugaacuuccccuccgacggccccguaaugcagaagaagacucugggcugggagcccuccaccgagcgccuguacccccgcgacggcgugcugaagggcgagauccacaaggcgcugaagcugaagggcggcggccacuaccugguggaguucaagucaaucuacauggccaagaagcccgugaagcugcccggcuacuacuacguggacuccaagcuggacaucaccucccacaacgaggacuacaccgugguggagcaguacgagcgcgccgaggcccgccaccaccuguuccaguaggguaccgagcucggauccacuaguccagugugguggaauucguucacugccguauaggcagcgagacgagcuugcgucucgguuuuagagcuagaaauagcaaguuaaaauaaggcuaguccguuaucaacuugaaaaaguggcaccgagucggugcguucacugccguauaggcagcggccgcgucgacaaucaaccucuggauuacaaaauuugugaaagauugacugguauucuuaacuauguugcuccuuuuacgcuauguggauacgcugcuuuaaugccuuuguaucaugcuauugcuucccguauggcuuucauuuucuccuccuuguauaaauccugguugcugucucuuuaugaggaguuguggcccguugucaggcaacguggcguggugugcacuguguuugcugacgcaacccccacugguuggggcauugccaccaccugucagcuccuuuccgggacuuucgcuuucccccucccuauugccacggcggaacucaucgccgccugccuugcccgcugcuggacaggggcucggcuguugggcacugacaauuccgugguguugucucgaaacccgcugaucagccucgacugugccuucuaguugccagccaucuguuguuugccccucccccgugccuuccuugacccuggaaggugccacucccacuguccuuuccuaauaaaaugaggaaauugcaucgca

SEQ ID NO: 81 - DNA, 1578 bp, artificial sequence
  DNA sequence encoding pre-C4/C9-stuffer sgRNA
gtcagatcgcctgcagacgccatccacgctgttttgacctccatagaagacaccgggaccgatccagcctccgcggccgggaacggtgcattggaacgcggattccccgtgccaagagtgactcaccgtccttgacacgaagcttgctagcgctaccggactcagatccaccggtcgccaccatggatagcactgagaacgtcatcaagcccttcatgcgcttcaaggtgcacatggagggctccgtgaacggccacgagttcgagatcgagggcgagggcgagggcaagccctacgagggcacccagaccgccaagctgcaggtgaccaagggcggccccctgcccttcgcctgggacatcctgtccccccagttccagtacggctccaaggtgtacgtgaagcaccccgccgacatccccgactacaagaagctgtccttccccgagggcttcaagtgggagcgcgtgatgaacttcgaggacggcggcgtggtgaccgtgacccaggactcctccctgcaggacggcaccttcatctaccacgtgaagttcatcggcgtgaacttcccctccgacggccccgtaatgcagaagaagactctgggctgggagccctccaccgagcgcctgtacccccgcgacggcgtgctgaagggcgagatccacaaggcgctgaagctgaagggcggcggccactacctggtggagttcaagtcaatctacatggccaagaagcccgtgaagctgcccggctactactacgtggactccaagctggacatcacctcccacaacgaggactacaccgtggtggagcagtacgagcgcgccgaggcccgccaccacctgttccagtagggtaccgagctcggatccactagtccagtgtggtggaattcgttcactgccgtataggcagcgagacgagcttgcgtctcggttttagagctagaaatagcaagttaaaataaggctagtccgttatcaacttgaaaaagtggcaccgagtcggtgcgttcactgccgtataggcagcggccgcgtcgacaatcaacctctggattacaaaatttgtgaaagattgactggtattcttaactatgttgctccttttacgctatgtggatacgctgctttaatgcctttgtatcatgctattgcttcccgtatggctttcattttctcctccttgtataaatcctggttgctgtctctttatgaggagttgtggcccgttgtcaggcaacgtggcgtggtgtgcactgtgtttgctgacgcaacccccactggttggggcattgccaccacctgtcagctcctttccgggactttcgctttccccctccctattgccacggcggaactcatcgccgcctgccttgcccgctgctggacaggggctcggctgttgggcactgacaattccgtggtgttgtctcgaaacccgctgatcagcctcgactgtgccttctagttgccagccatctgttgtttgcccctcccccgtgccttccttgaccctggaaggtgccactcccactgtcctttcctaataaaatgaggaaattgcatcgca

SEQ ID NO: 82 - RNA, 1695 nt, artificial sequence
  pre-C4/C9-gfp c.187 A>G sgRNA
gucagaucgccugcagacgccauccacgcuguuuugaccuccauagaagacaccgggaccgauccagccuccgcggccgggaacggugcauuggaacgcggauuccccgugccaagagugacucaccguccuugacacgaagcuugcuagcgcuaccggacucagauccaccggucgccaccauggauagcacugagaacgucaucaagcccuucaugcgcuucaaggugcacauggagggcuccgugaacggccacgaguucgagaucgagggcgagggcgagggcaagcccuacgagggcacccagaccgccaagcugcaggugaccaagggcggcccccugcccuucgccugggacauccuguccccccaguuccaguacggcuccaagguguacgugaagcaccccgccgacauccccgacuacaagaagcuguccuuccccgagggcuucaagugggagcgcgugaugaacuucgaggacggcggcguggugaccgugacccaggacuccucccugcaggacggcaccuucaucuaccacgugaaguucaucggcgugaacuuccccuccgacggccccguaaugcagaagaagacucugggcugggagcccuccaccgagcgccuguacccccgcgacggcgugcugaagggcgagauccacaaggcgcugaagcugaagggcggcggccacuaccugguggaguucaagucaaucuacauggccaagaagcccgugaagcugcccggcuacuacuacguggacuccaagcuggacaucaccucccacaacgaggacuacaccgugguggagcaguacgagcgcgccgaggcccgccaccaccuguuccaguaggguaccgagcucggauccacuaguccagugugguggaauucguucacugccguauaggcaggccguaggucaggguggucacgguuuuagagcuagaaauagcaaguuaaaauaaggcuaguccguuaucaacuugaaaaaguggcaccgagucggugcguucacugccguauaggcacagggucagcuugccguaggguuuuagagcuagaaauagcaaguuaaaauaaggcuaguccguuaucaacuugaaaaaguggcaccgagucggugcguucacugccguauaggcagcggccgcgucgacaaucaaccucuggauuacaaaauuugugaaagauugacugguauucuuaacuauguugcuccuuuuacgcuauguggauacgcugcuuuaaugccuuuguaucaugcuauugcuucccguauggcuuucauuuucuccuccuuguauaaauccugguugcugucucuuuaugaggaguuguggcccguugucaggcaacguggcguggugugcacuguguuugcugacgcaacccccacugguuggggcauugccaccaccugucagcuccuuuccgggacuuucgcuuucccccucccuauugccacggcggaacucaucgccgccugccuugcccgcugcuggacaggggcucggcuguugggcacugacaauuccgugguguugucucgaaacccgcugaucagccucgacugugccuucuaguugccagccaucuguuguuugccccucccccgugccuuccuugacccuggaaggugccacucccacuguccuuuccuaauaaaaugaggaaauugcaucgca

SEQ ID NO: 83 - DNA, 1695 bp, artificial sequence
  DNA sequence encoding pre-C4/C9-gfp c.187 A>G sgRNA
gtcagatcgcctgcagacgccatccacgctgttttgacctccatagaagacaccgggaccgatccagcctccgcggccgggaacggtgcattggaacgcggattccccgtgccaagagtgactcaccgtccttgacacgaagcttgctagcgctaccggactcagatccaccggtcgccaccatggatagcactgagaacgtcatcaagcccttcatgcgcttcaaggtgcacatggagggctccgtgaacggccacgagttcgagatcgagggcgagggcgagggcaagccctacgagggcacccagaccgccaagctgcaggtgaccaagggcggccccctgcccttcgcctgggacatcctgtccccccagttccagtacggctccaaggtgtacgtgaagcaccccgccgacatccccgactacaagaagctgtccttccccgagggcttcaagtgggagcgcgtgatgaacttcgaggacggcggcgtggtgaccgtgacccaggactcctccctgcaggacggcaccttcatctaccacgtgaagttcatcggcgtgaacttcccctccgacggccccgtaatgcagaagaagactctgggctgggagccctccaccgagcgcctgtacccccgcgacggcgtgctgaagggcgagatccacaaggcgctgaagctgaagggcggcggccactacctggtggagttcaagtcaatctacatggccaagaagcccgtgaagctgcccggctactactacgtggactccaagctggacatcacctcccacaacgaggactacaccgtggtggagcagtacgagcgcgccgaggcccgccaccacctgttccagtagggtaccgagctcggatccactagtccagtgtggtggaattcgttcactgccgtataggcaggccgtaggtcagggtggtcacggttttagagctagaaatagcaagttaaaataaggctagtccgttatcaacttgaaaaagtggcaccgagtcggtgcgttcactgccgtataggcacagggtcagcttgccgtagggttttagagctagaaatagcaagttaaaataaggctagtccgttatcaacttgaaaaagtggcaccgagtcggtgcgttcactgccgtataggcagcggccgcgtcgacaatcaacctctggattacaaaatttgtgaaagattgactggtattcttaactatgttgctccttttacgctatgtggatacgctgctttaatgcctttgtatcatgctattgcttcccgtatggctttcattttctcctccttgtataaatcctggttgctgtctctttatgaggagttgtggcccgttgtcaggcaacgtggcgtggtgtgcactgtgtttgctgacgcaacccccactggttggggcattgccaccacctgtcagctcctttccgggactttcgctttccccctccctattgccacggcggaactcatcgccgcctgccttgcccgctgctggacaggggctcggctgttgggcactgacaattccgtggtgttgtctcgaaacccgctgatcagcctcgactgtgccttctagttgccagccatctgttgtttgcccctcccccgtgccttccttgaccctggaaggtgccactcccactgtcctttcctaataaaatgaggaaattgcatcgca

SEQ ID NO: 84 - protein, 19 aa, artificial sequence
  P2A peptide
ATNFSLLKQAGDVEENPGP

SEQ ID NO: 85 - protein, 20 aa, artificial sequence
  E2A peptide
QCTNYALLKLAGDVESNPGP

SEQ ID NO: 86 - protein, 22 aa, artificial sequence
  F2A peptide
VKQTLNFDLLKLAGDVESNPGP